European Patent Specification EP 3 735 478 B1, published August 16, 2023. Title: MUTANT AND GENETICALLY MODIFIED BACILLUS CELLS AND METHODS THEREOF FOR INCREASED PROTEIN PRODUCTION. Applicant: DANISCO. The sequence listing filed with the application follows.

SEQUENCE LISTING (84 sequences)

SEQ ID NO: 1 - DNA, 4188 bp, Artificial Sequence
  synthetic polynucleotide encoding Cas9
gtggccccaaaaaagaaacgcaaggttatggataaaaaatacagcattggtctggatatcggaaccaacagcgttgggtgggcagtaataacagatgaatacaaagtgccgtcaaaaaaatttaaggttctggggaatacagatcgccacagcataaaaaagaatctgattggggcattgctgtttgattcgggtgagacagctgaggccacgcgtctgaaacgtacagcaagaagacgttacacacgtcgtaaaaatcgtatttgctacttacaggaaattttttctaacgaaatggccaaggtagatgatagtttcttccatcgtctcgaagaatcttttctggttgaggaagataaaaaacacgaacgtcaccctatctttggcaatatcgtggatgaagtggcctatcatgaaaaataccctacgatttatcatcttcgcaagaagttggttgatagtacggacaaagcggatctgcgtttaatctatcttgcgttagcgcacatgatcaaatttcgtggtcatttcttaattgaaggtgatctgaatcctgataactctgatgtggacaaattgtttatacaattagtgcaaacctataatcagctgttcgaggaaaaccccattaatgcctctggagttgatgccaaagcgattttaagcgcgagactttctaagtcccggcgtctggagaatctgatcgcccagttaccaggggaaaagaaaaatggtctgtttggtaatctgattgccctcagtctggggcttaccccgaacttcaaatccaattttgacctggctgaggacgcaaagctgcagctgagcaaagatacttatgatgatgacctcgacaatctgctcgcccagattggtgaccaatatgcggatctgtttctggcagcgaagaatctttcggatgctatcttgctgtcggatattctgcgtgttaataccgaaatcaccaaagcgcctctgtctgcaagtatgatcaagagatacgacgagcaccaccaggacctgactcttcttaaggcactggtacgccaacagcttccggagaaatacaaagaaatattcttcgaccagtccaagaatggttacgcgggctacatcgatggtggtgcatcacaggaagagttctataaatttattaaaccaatccttgagaaaatggatggcacggaagagttacttgttaaacttaaccgcgaagacttgcttagaaagcaacgtacattcgacaacggctccatcccacaccagattcatttaggtgaacttcacgccatcttgcgcagacaagaagatttctatcccttcttaaaagacaatcgggagaaaatcgagaagatcctgacgttccgcattccctattatgtcggtcccctggcacgtggtaattctcggtttgcctggatgacgcgcaaaagtgaggaaaccatcaccccttggaactttgaagaagtcgtggataaaggtgctagcgcgcagtcttttatagaaagaatgacgaacttcgataaaaacttgcccaacgaaaaagtcctgcccaagcactctcttttatatgagtactttactgtgtacaacgaactgactaaagtgaaatacgttacggaaggtatgcgcaaacctgcctttcttagtggcgagcagaaaaaagcaattgtcgatcttctctttaaaacgaatcgcaaggtaactgtaaaacagctgaaggaagattatttcaaaaagatcgaatgctttgattctgtcgagatctcgggtgtcgaagatcgtttcaacgcttccttagggacctatcatgatttgctgaagataataaaagacaaagactttctcgacaatgaagaaaatgaagatattctggaggatattgttttgaccttgaccttattcgaagatagagagatgatcgaggagcgcttaaaaacctatgcccacctgtttgatgacaaagtcatgaagcaattaaagcgccgcagatatacggggtggggccgcttgagccgcaagttgattaacggtattagagacaagcagagcggaaaaactatcctggatttcctcaaatctgacggatttgcgaaccgcaattttatgcagcttatacatgatgattcgcttacattcaaagaggatattcagaaggctcaggtgtctgggcaaggtgattcactccacgaacatatagcaaatttggccggctctcctgcgattaagaaggggatcctgcaaacagttaaagttgtggatgaacttgtaaaagtaatgggccgccacaagccggagaatatcgtgatagaaatggcgcgcgagaatcaaacgacacaaaaaggtcaaaagaactcaagagagagaatgaagcgcattgaggaggggataaaggaacttggatctcaaattctgaaagaacatccagttgaaaacactcagctgcaaaatgaaaaattgtacctgtactacctgcagaatggaagagacatgtacgtggatcaggaattggatatcaatagactctcggactatgacgtagatcacattgtccctcagagcttcctcaaggatgattctatagataataaagtacttacgagatcggacaaaaatcgcggtaaatcggataacgtcccatcggaggaagtcgttaaaaagatgaaaaactattggcgtcaactgctgaacgccaagctgatcacacagcgtaagtttgataatctgactaaagccgaacgcggtggtcttagtgaactcgataaagcaggatttataaaacggcagttagtagaaacgcgccaaattacgaaacacgtggctcagatcctcgattctagaatgaatacaaagtacgatgaaaacgataaactgatccgtgaagtaaaagtcattaccttaaaatctaaacttgtgtccgatttccgcaaagattttcagttttacaaggtccgggaaatcaataactatcaccatgcacatgatgcatatttaaatgcggttgtaggcacggcccttattaagaaataccctaaactcgaaagtgagtttgtttatggggattataaagtgtatgacgttcgcaaaatgatcgcgaaatcagaacaggaaatcggtaaggctaccgctaaatactttttttattccaacattatgaatttttttaagaccgaaataactctcgcgaatggtgaaatccgtaaacggcctcttatagaaaccaatggtgaaacgggagaaatcgtttgggataaaggtcgtgactttgccaccgttcgtaaagtcctctcaatgccgcaagttaacattgtcaagaagacggaagttcaaacagggggattctccaaagaatctatcctgccgaagcgtaacagtgataaacttattgccagaaaaaaagattgggatccaaaaaaatacggaggctttgattcccctaccgtcgcgtatagtgtgctggtggttgctaaagtcgagaaagggaaaagcaagaaattgaaatcagttaaagaactgctgggtattacaattatggaaagatcgtcctttgagaaaaatccgatcgactttttagaggccaaggggtataaggaagtgaaaaaagatctcatcatcaaattaccgaagtatagtctttttgagctggaaaacggcagaaaaagaatgctggcctccgcgggcgagttacagaagggaaatgagctggcgctgccttccaaatatgttaattttctgtaccttgccagtcattatgagaaactgaagggcagccccgaagataacgaacagaaacaattattcgtggaacagcataagcactatttagatgaaattatagagcaaattagtgaattttctaagcgcgttatcctcgcggatgctaatttagacaaagtactgtcagcttataataaacatcgggataagccgattagagaacaggccgaaaatatcattcatttgtttaccttaaccaaccttggagcaccagctgccttcaaatatttcgataccacaattgatcgtaaacggtatacaagtacaaaagaagtcttggacgcaaccctcattcatcaatctattactggattatatgagacacgcattgatctttcacagctgggcggagacaagaagaaaaaactgaaactgcaccatcatcaccatcatcatcaccatcattgataa

SEQ ID NO: 2 - protein, 8 aa, Artificial Sequence
  N-terminal NLS
APKKKRKV

SEQ ID NO: 3 - protein, 6 aa, Artificial Sequence
  C-terminal NLS
KKKKLK

SEQ ID NO: 4 - protein, 10 aa, Artificial Sequence
  10-histidine tag
HHHHHHHHHH

SEQ ID NO: 5 - DNA, 607 bp, Bacillus subtilis
attcctccattttcttctgctatcaaaataacagactcgtgattttccaaacgagctttcaaaaaagcctctgccccttgcaaatcggatgcctgtctataaaattcccgatattggttaaacagcggcgcaatggcggccgcatctgatgtctttgcttggcgaatgttcatcttatttcttcctccctctcaataattttttcattctatcccttttctgtaaagtttatttttcagaatacttttatcatcatgctttgaaaaaatatcacgataatatccattgttctcacggaagcacacgcaggtcatttgaacgaattttttcgacaggaatttgccgggactcaggagcatttaacctaaaaaagcatgacatttcagcataatgaacatttactcatgtctattttcgttcttttctgtatgaaaatagttatttcgagtctctacggaaatagcgagagatgatatacctaaatagagataaaatcatctcaaaaaaatgggtctactaaaatattattccatctattacaataaattcacagaatagtcttttaagtaagtctactctgaatttttttaaaaggagagggtaacta

SEQ ID NO: 6 - DNA, 50 bp, Artificial Sequence
  Cas9 forward primer
atatatgagtaaacttggtctgacagaattcctccattttcttctgctat

SEQ ID NO: 7 - DNA, 35 bp, Artificial Sequence
  Cas9 reverse primer
tgcggccgcgaattcgattacgaatgccgtctccc

SEQ ID NO: 8 - DNA, 3290 bp, Artificial Sequence
  pKB320 backbone
gaattcgcggccgcacgcgtccatggggatccccgcgggtcgacctcgagagttacgctagggataacagggtaatataggagctccagtcggcttaaaccagttttcgctggtgcgaaaaaagagtgtcttgtgacacctaaattcaaaatctatcggtcagatttataccgatttgattttatatattcttgaataacatacgccgagttatcacataaaagcgggaaccaatcataaaatttaaacttcattgcataatccattaaactcttaaattctacgattccttgttcatcaataaactcaatcatttctttaattaatttatatctatctgttgttgttttctttaataattcattaacatctacaccgccataaactatcatatcttctttttgatatttaaatttattaggatcgtccatgtgaagcatatatctcacaagacctttcacacttcctgcaatctgcggaatagtcgcattcaattcttctgttaattatttttatctgttcataagatttattaccctcatacatcactagaatatgataatgctcttttttcatcctaccttctgtatcagtatccctatcatgtaatggagacactacaaattgaatgtgtaactcttttaaatactctaaccactcggcttttgctgattctggatataaaacaaatgtccaattacgtcctcttgaatttttcttgttttcagtttcttttattacattttcgctcatgatataataacggtgctaatacacttaacaaaatttagtcatagataggcagcatgccagtgctgtctatctttttttgtttaaaatgcaccgtattcctcctttgcatatttttttattagaataccggttgcatctgatttgctaatattatatttttctttgattctatttaatatctcattttcttctgttgtaagtcttaaagtaacagcaacttttttctcttcttttctatctacaactatcactgtacctcccaacatctgtttttttcactttaacataaaaaacaaccttttaacattaaaaacccaatatttatttatttgtttggacaatggacactggacacctaggggggaggtcgtagtacccccctatgttttctcccctaaataaccccaaaaatctaagaaaaaaagacctcaaaaaggtctttaattaacatctcaaatttcgcatttattccaatttcctttttgcgtgtgatgcgagctcatcggctccgtcgatactatgttatacgccaactttcaaaacaactttgaaaaagctgttttctggtatttaaggttttagaatgcaaggaacagtgaattggagttcgtcttgttataattagcttcttggggtatctttaaatactgtagaaaagaggaaggaaataataaatggctaaaatgagaatatcaccggaattgaaaaaactgatcgaaaaataccgctgcgtaaaagatacggaaggaatgtctcctgctaaggtatataagctggtgggagaaaatgaaaacctatatttaaaaatgacggacagccggtataaagggaccacctatgatgtggaacgggaaaaggacatgatgctatggctggaaggaaagctgcctgttccaaaggtcctgcactttgaacggcatgatggctggagcaatctgctcatgagtgaggccgatggcgtcctttgctcggaagagtatgaagatgaacaaagccctgaaaagattatcgagctgtatgcggagtgcatcaggctctttcactccatcgacatatcggattgtccctatacgaatagcttagacagccgcttagccgaattggattacttactgaataacgatctggccgatgtggattgcgaaaactgggaagaagacactccatttaaagatccgcgcgagctgtatgattttttaaagacggaaaagcccgaagaggaacttgtcttttcccacggcgacctgggagacagcaacatctttgtgaaagatggcaaagtaagtggctttattgatcttgggagaagcggcagggcggacaagtggtatgacattgccttctgcgtccggtcgatcagggaggatatcggggaagaacagtatgtcgagctattttttgacttactggggatcaagcctgattgggagaaaataaaatattatattttactggatgaattgttttagtgactgcagtgagatctggtaatgactctctagcttgaggcatcaaataaaacgaaaggctcagtcgaaagactgggcctttcgttttatctgttgtttgtcggtgaacgctctcctgagtaggacaaatccgccgctctagctaagcagaaggccatcctgacggatggcctttttgcgtttctacaaactcttgttaactctagagctgcctgccgcgtttcggtgatgaagatcttcccgatgattaattaattcagaacgctcggttgccgccgggcgttttttatgaagcttcgttgctggcgtttttccataggctccgcccccctgacgagcatcacaaaaatcgacgctcaagtcagaggtggcgaaacccgacaggactataaagataccaggcgtttccccctggaagctccctcgtgcgctctcctgttccgaccctgccgcttaccggatacctgtccgcctttctcccttcgggaagcgtggcgctttctcatagctcacgctgtaggtatctcagttcggtgtaggtcgttcgctccaagctgggctgtgtgcacgaaccccccgttcagcccgaccgctgcgccttatccggtaactatcgtcttgagtccaacccggtaagacacgacttatcgccactggcagcagccactggtaacaggattagcagagcgaggtatgtaggcggtgctacagagttcttgaagtggtggcctaactacggctacactagaaggacagtatttggtatctgcgctctgctgaagccagttaccttcggaaaaagagttggtagctcttgatccggcaaacaaaccaccgctggtagcggtggtttttttgtttgcaagcagcagattacgcgcagaaaaaaaggatctcaagaagatcctttgatcttttctacggggtctgacgctcagtggaacgaaaactcacgttaagggattttggtcatgagattatcaaaaaggatcttcacctagatccttttaaattaaaaatgaagttttaaatcaatctaaagtatatatgagtaaacttggtctgaca

SEQ ID NO: 9 - DNA, 4204 bp, Artificial Sequence
  pKB320
gcggccgcacgcgtccatggggatccccgcgggtcgacctcgagagttacgctagggataacagggtaatataggagctccagtcggcttaaaccagttttcgctggtgcgaaaaaagagtgtcttgtgacacctaaattcaaaatctatcggtcagatttataccgatttgattttatatattcttgaataacatacgccgagttatcacataaaagcgggaaccaatcataaaatttaaacttcattgcataatccattaaactcttaaattctacgattccttgttcatcaataaactcaatcatttctttaattaatttatatctatctgttgttgttttctttaataattcattaacatctacaccgccataaactatcatatcttctttttgatatttaaatttattaggatcgtccatgtgaagcatatatctcacaagacctttcacacttcctgcaatctgcggaatagtcgcattcaattcttctgttaattatttttatctgttcataagatttattaccctcatacatcactagaatatgataatgctcttttttcatcctaccttctgtatcagtatccctatcatgtaatggagacactacaaattgaatgtgtaactcttttaaatactctaaccactcggcttttgctgattctggatataaaacaaatgtccaattacgtcctcttgaatttttcttgttttcagtttcttttattacattttcgctcatgatataataacggtgctaatacacttaacaaaatttagtcatagataggcagcatgccagtgctgtctatctttttttgtttaaaatgcaccgtattcctcctttgcatatttttttattagaataccggttgcatctgatttgctaatattatatttttctttgattctatttaatatctcattttcttctgttgtaagtcttaaagtaacagcaacttttttctcttcttttctatctacaactatcactgtacctcccaacatctgtttttttcactttaacataaaaaacaaccttttaacattaaaaacccaatatttatttatttgtttggacaatggacactggacacctaggggggaggtcgtagtacccccctatgttttctcccctaaataaccccaaaaatctaagaaaaaaagacctcaaaaaggtctttaattaacatctcaaatttcgcatttattccaatttcctttttgcgtgtgatgcgagctcatcggctccgtcgatactatgttatacgccaactttcaaaacaactttgaaaaagctgttttctggtatttaaggttttagaatgcaaggaacagtgaattggagttcgtcttgttataattagcttcttggggtatctttaaatactgtagaaaagaggaaggaaataataaatggctaaaatgagaatatcaccggaattgaaaaaactgatcgaaaaataccgctgcgtaaaagatacggaaggaatgtctcctgctaaggtatataagctggtgggagaaaatgaaaacctatatttaaaaatgacggacagccggtataaagggaccacctatgatgtggaacgggaaaaggacatgatgctatggctggaaggaaagctgcctgttccaaaggtcctgcactttgaacggcatgatggctggagcaatctgctcatgagtgaggccgatggcgtcctttgctcggaagagtatgaagatgaacaaagccctgaaaagattatcgagctgtatgcggagtgcatcaggctctttcactccatcgacatatcggattgtccctatacgaatagcttagacagccgcttagccgaattggattacttactgaataacgatctggccgatgtggattgcgaaaactgggaagaagacactccatttaaagatccgcgcgagctgtatgattttttaaagacggaaaagcccgaagaggaacttgtcttttcccacggcgacctgggagacagcaacatctttgtgaaagatggcaaagtaagtggctttattgatcttgggagaagcggcagggcggacaagtggtatgacattgccttctgcgtccggtcgatcagggaggatatcggggaagaacagtatgtcgagctattttttgacttactggggatcaagcctgattgggagaaaataaaatattatattttactggatgaattgttttagtgactgcagtgagatctggtaatgactctctagcttgaggcatcaaataaaacgaaaggctcagtcgaaagactgggcctttcgttttatctgttgtttgtcggtgaacgctctcctgagtaggacaaatccgccgctctagctaagcagaaggccatcctgacggatggcctttttgcgtttctacaaactcttgttaactctagagctgcctgccgcgtttcggtgatgaagatcttcccgatgattaattaattcagaacgctcggttgccgccgggcgttttttatgaagcttcgttgctggcgtttttccataggctccgcccccctgacgagcatcacaaaaatcgacgctcaagtcagaggtggcgaaacccgacaggactataaagataccaggcgtttccccctggaagctccctcgtgcgctctcctgttccgaccctgccgcttaccggatacctgtccgcctttctcccttcgggaagcgtggcgctttctcatagctcacgctgtaggtatctcagttcggtgtaggtcgttcgctccaagctgggctgtgtgcacgaaccccccgttcagcccgaccgctgcgccttatccggtaactatcgtcttgagtccaacccggtaagacacgacttatcgccactggcagcagccactggtaacaggattagcagagcgaggtatgtaggcggtgctacagagttcttgaagtggtggcctaactacggctacactagaaggacagtatttggtatctgcgctctgctgaagccagttaccttcggaaaaagagttggtagctcttgatccggcaaacaaaccaccgctggtagcggtggtttttttgtttgcaagcagcagattacgcgcagaaaaaaaggatctcaagaagatcctttgatcttttctacggggtctgacgctcagtggaacgaaaactcacgttaagggattttggtcatgagattatcaaaaaggatcttcacctagatccttttaaattaaaaatgaagttttaaatcaatctaaagtatatatgagtaaacttggtctgacagttaccaatgcttaatcagtgaggcacctatctcagcgatctgtctatttcgttcatccatagttgcctgactccccgtcgtgtagataactacgatacgggagggcttaccatctggccccagtgctgcaatgataccgcgagacccacgctcaccggctccagatttatcagcaataaaccagccagccggaagggccgagcgcagaagtggtcctgcaactttatccgcctccatccagtctattaattgttgccgggaagctagagtaagtagttcgccagttaatagtttgcgcaacgttgttgccattgctacaggcatcgtggtgtcacgctcgtcgtttggtatggcttcattcagctccggttcccaacgatcaaggcgagttacatgatcccccatgttgtgcaaaaaagcggttagctccttcggtcctccgatcgttgtcagaagtaagttggccgcagtgttatcactcatggttatggcagcactgcataattctcttactgtcatgccatccgtaagatgcttttctgtgactggtgagtactcaaccaagtcattctgagaatagtgtatgcggcgaccgagttgctcttgcccggcgtcaatacgggataataccgcgccacatagcagaactttaaaagtgctcatcattggaaaacgttcttcggggcgaaaactctcaaggatcttaccgctgttgagatccagttcgatgtaacccactcgtgcacccaactgatcttcagcatcttttactttcaccagcgtttctgggtgagcaaaaacaggaaggcaaaatgccgcaaaaaagggaataagggcgacacggaaatgttgaatactcatactcttcctttttcaatattattgaagcatttatcagggttattgtctcatggaattc

SEQ ID NO: 10 - DNA, 35 bp, Artificial Sequence
  pKB320 forward primer
gggagacggcattcgtaatcgaattcgcggccgca

SEQ ID NO: 11 - DNA, 50 bp, Artificial Sequence
  pKB320 reverse primer
atagcagaagaaaatggaggaattctgtcagaccaagtttactcatatat

SEQ ID NO: 12 - DNA, 23 bp, Artificial Sequence
  Cas9 reverse sequencing primer
ccgactggagctcctatattacc

SEQ ID NO: 13 - DNA, 20 bp, Artificial Sequence
  Cas9 reverse sequening primer 2
gctgtggcgatctgtattcc

SEQ ID NO: 14 - DNA, 22 bp, Artificial Sequence
  Cas9 forward sequencing primer 1
gtcttttaagtaagtctactct

SEQ ID NO: 15 - DNA, 20 bp, Artificial Sequence
  Cas9 forward seq primer 2
ccaaagcgattttaagcgcg

SEQ ID NO: 16 - DNA, 20 bp, Artificial Sequence
  Cas9 forward seq primer 3
cctggcacgtggtaattctc

SEQ ID NO: 17 - DNA, 20 bp, Artificial Sequence
  Cas9 forward seq primer 4
ggatttcctcaaatctgacg

SEQ ID NO: 18 - DNA, 21 bp, Artificial Sequence
  Cas9 forward seq primer 5
gtagaaacgcgccaaattacg

SEQ ID NO: 19 - DNA, 20 bp, Artificial Sequence
  Cas9 forward seq primer 6
gctggtggttgctaaagtcg

SEQ ID NO: 20 - DNA, 20 bp, Artificial Sequence
  Cas9 forward seq primer 7
ggacgcaaccctcattcatc

SEQ ID NO: 21 - DNA, 8347 bp, Artificial Sequence
  pRF694
gaattcctccattttcttctgctatcaaaataacagactcgtgattttccaaacgagctttcaaaaaagcctctgccccttgcaaatcggatgcctgtctataaaattcccgatattggttaaacagcggcgcaatggcggccgcatctgatgtctttgcttggcgaatgttcatcttatttcttcctccctctcaataattttttcattctatcccttttctgtaaagtttatttttcagaatacttttatcatcatgctttgaaaaaatatcacgataatatccattgttctcacggaagcacacgcaggtcatttgaacgaattttttcgacaggaatttgccgggactcaggagcatttaacctaaaaaagcatgacatttcagcataatgaacatttactcatgtctattttcgttcttttctgtatgaaaatagttatttcgagtctctacggaaatagcgagagatgatatacctaaatagagataaaatcatctcaaaaaaatgggtctactaaaatattattccatctattacaataaattcacagaatagtcttttaagtaagtctactctgaatttttttaaaaggagagggtaactagtggccccaaaaaagaaacgcaaggttatggataaaaaatacagcattggtctggatatcggaaccaacagcgttgggtgggcagtaataacagatgaatacaaagtgccgtcaaaaaaatttaaggttctggggaatacagatcgccacagcataaaaaagaatctgattggggcattgctgtttgattcgggtgagacagctgaggccacgcgtctgaaacgtacagcaagaagacgttacacacgtcgtaaaaatcgtatttgctacttacaggaaattttttctaacgaaatggccaaggtagatgatagtttcttccatcgtctcgaagaatcttttctggttgaggaagataaaaaacacgaacgtcaccctatctttggcaatatcgtggatgaagtggcctatcatgaaaaataccctacgatttatcatcttcgcaagaagttggttgatagtacggacaaagcggatctgcgtttaatctatcttgcgttagcgcacatgatcaaatttcgtggtcatttcttaattgaaggtgatctgaatcctgataactctgatgtggacaaattgtttatacaattagtgcaaacctataatcagctgttcgaggaaaaccccattaatgcctctggagttgatgccaaagcgattttaagcgcgagactttctaagtcccggcgtctggagaatctgatcgcccagttaccaggggaaaagaaaaatggtctgtttggtaatctgattgccctcagtctggggcttaccccgaacttcaaatccaattttgacctggctgaggacgcaaagctgcagctgagcaaagatacttatgatgatgacctcgacaatctgctcgcccagattggtgaccaatatgcggatctgtttctggcagcgaagaatctttcggatgctatcttgctgtcggatattctgcgtgttaataccgaaatcaccaaagcgcctctgtctgcaagtatgatcaagagatacgacgagcaccaccaggacctgactcttcttaaggcactggtacgccaacagcttccggagaaatacaaagaaatattcttcgaccagtccaagaatggttacgcgggctacatcgatggtggtgcatcacaggaagagttctataaatttattaaaccaatccttgagaaaatggatggcacggaagagttacttgttaaacttaaccgcgaagacttgcttagaaagcaacgtacattcgacaacggctccatcccacaccagattcatttaggtgaacttcacgccatcttgcgcagacaagaagatttctatcccttcttaaaagacaatcgggagaaaatcgagaagatcctgacgttccgcattccctattatgtcggtcccctggcacgtggtaattctcggtttgcctggatgacgcgcaaaagtgaggaaaccatcaccccttggaactttgaagaagtcgtggataaaggtgctagcgcgcagtcttttatagaaagaatgacgaacttcgataaaaacttgcccaacgaaaaagtcctgcccaagcactctcttttatatgagtactttactgtgtacaacgaactgactaaagtgaaatacgttacggaaggtatgcgcaaacctgcctttcttagtggcgagcagaaaaaagcaattgtcgatcttctctttaaaacgaatcgcaaggtaactgtaaaacagctgaaggaagattatttcaaaaagatcgaatgctttgattctgtcgagatctcgggtgtcgaagatcgtttcaacgcttccttagggacctatcatgatttgctgaagataataaaagacaaagactttctcgacaatgaagaaaatgaagatattctggaggatattgttttgaccttgaccttattcgaagatagagagatgatcgaggagcgcttaaaaacctatgcccacctgtttgatgacaaagtcatgaagcaattaaagcgccgcagatatacggggtggggccgcttgagccgcaagttgattaacggtattagagacaagcagagcggaaaaactatcctggatttcctcaaatctgacggatttgcgaaccgcaattttatgcagcttatacatgatgattcgcttacattcaaagaggatattcagaaggctcaggtgtctgggcaaggtgattcactccacgaacatatagcaaatttggccggctctcctgcgattaagaaggggatcctgcaaacagttaaagttgtggatgaacttgtaaaagtaatgggccgccacaagccggagaatatcgtgatagaaatggcgcgcgagaatcaaacgacacaaaaaggtcaaaagaactcaagagagagaatgaagcgcattgaggaggggataaaggaacttggatctcaaattctgaaagaacatccagttgaaaacactcagctgcaaaatgaaaaattgtacctgtactacctgcagaatggaagagacatgtacgtggatcaggaattggatatcaatagactctcggactatgacgtagatcacattgtccctcagagcttcctcaaggatgattctatagataataaagtacttacgagatcggacaaaaatcgcggtaaatcggataacgtcccatcggaggaagtcgttaaaaagatgaaaaactattggcgtcaactgctgaacgccaagctgatcacacagcgtaagtttgataatctgactaaagccgaacgcggtggtcttagtgaactcgataaagcaggatttataaaacggcagttagtagaaacgcgccaaattacgaaacacgtggctcagatcctcgattctagaatgaatacaaagtacgatgaaaacgataaactgatccgtgaagtaaaagtcattaccttaaaatctaaacttgtgtccgatttccgcaaagattttcagttttacaaggtccgggaaatcaataactatcaccatgcacatgatgcatatttaaatgcggttgtaggcacggcccttattaagaaataccctaaactcgaaagtgagtttgtttatggggattataaagtgtatgacgttcgcaaaatgatcgcgaaatcagaacaggaaatcggtaaggctaccgctaaatactttttttattccaacattatgaatttttttaagaccgaaataactctcgcgaatggtgaaatccgtaaacggcctcttatagaaaccaatggtgaaacgggagaaatcgtttgggataaaggtcgtgactttgccaccgttcgtaaagtcctctcaatgccgcaagttaacattgtcaagaagacggaagttcaaacagggggattctccaaagaatctatcctgccgaagcgtaacagtgataaacttattgccagaaaaaaagattgggatccaaaaaaatacggaggctttgattcccctaccgtcgcgtatagtgtgctggtggttgctaaagtcgagaaagggaaaagcaagaaattgaaatcagttaaagaactgctgggtattacaattatggaaagatcgtcctttgagaaaaatccgatcgactttttagaggccaaggggtataaggaagtgaaaaaagatctcatcatcaaattaccgaagtatagtctttttgagctggaaaacggcagaaaaagaatgctggcctccgcgggcgagttacagaagggaaatgagctggcgctgccttccaaatatgttaattttctgtaccttgccagtcattatgagaaactgaagggcagccccgaagataacgaacagaaacaattattcgtggaacagcataagcactatttagatgaaattatagagcaaattagtgaattttctaagcgcgttatcctcgcggatgctaatttagacaaagtactgtcagcttataataaacatcgggataagccgattagagaacaggccgaaaatatcattcatttgtttaccttaaccaaccttggagcaccagctgccttcaaatatttcgataccacaattgatcgtaaacggtatacaagtacaaaagaagtcttggacgcaaccctcattcatcaatctattactggattatatgagacacgcattgatctttcacagctgggcggagacaagaagaaaaaactgaaactgcaccatcatcaccatcatcatcaccatcattgataactcgagaaagcttacataaaaaaccggccttggccccgccggttttttattatttttcttcctccgcatgttcaatccgctccataatcgacggatggctccctctgaaaattttaacgagaaacggcgggttgacccggctcagtcccgtaacggccaagtcctgaaacgtctcaatcgccgcttcccggtttccggtcagctcaatgccgtaacggtcggcggcgttttcctgataccgggagacggcattcgtaatcgaattcgcggccgcacgcgtccatggggatccccgcgggtcgacctcgagagttacgctagggataacagggtaatataggagctccagtcggcttaaaccagttttcgctggtgcgaaaaaagagtgtcttgtgacacctaaattcaaaatctatcggtcagatttataccgatttgattttatatattcttgaataacatacgccgagttatcacataaaagcgggaaccaatcataaaatttaaacttcattgcataatccattaaactcttaaattctacgattccttgttcatcaataaactcaatcatttctttaattaatttatatctatctgttgttgttttctttaataattcattaacatctacaccgccataaactatcatatcttctttttgatatttaaatttattaggatcgtccatgtgaagcatatatctcacaagacctttcacacttcctgcaatctgcggaatagtcgcattcaattcttctgttaattatttttatctgttcataagatttattaccctcatacatcactagaatatgataatgctcttttttcatcctaccttctgtatcagtatccctatcatgtaatggagacactacaaattgaatgtgtaactcttttaaatactctaaccactcggcttttgctgattctggatataaaacaaatgtccaattacgtcctcttgaatttttcttgttttcagtttcttttattacattttcgctcatgatataataacggtgctaatacacttaacaaaatttagtcatagataggcagcatgccagtgctgtctatctttttttgtttaaaatgcaccgtattcctcctttgcatatttttttattagaataccggttgcatctgatttgctaatattatatttttctttgattctatttaatatctcattttcttctgttgtaagtcttaaagtaacagcaacttttttctcttcttttctatctacaactatcactgtacctcccaacatctgtttttttcactttaacataaaaaacaaccttttaacattaaaaacccaatatttatttatttgtttggacaatggacactggacacctaggggggaggtcgtagtacccccctatgttttctcccctaaataaccccaaaaatctaagaaaaaaagacctcaaaaaggtctttaattaacatctcaaatttcgcatttattccaatttcctttttgcgtgtgatgcgagctcatcggctccgtcgatactatgttatacgccaactttcaaaacaactttgaaaaagctgttttctggtatttaaggttttagaatgcaaggaacagtgaattggagttcgtcttgttataattagcttcttggggtatctttaaatactgtagaaaagaggaaggaaataataaatggctaaaatgagaatatcaccggaattgaaaaaactgatcgaaaaataccgctgcgtaaaagatacggaaggaatgtctcctgctaaggtatataagctggtgggagaaaatgaaaacctatatttaaaaatgacggacagccggtataaagggaccacctatgatgtggaacgggaaaaggacatgatgctatggctggaaggaaagctgcctgttccaaaggtcctgcactttgaacggcatgatggctggagcaatctgctcatgagtgaggccgatggcgtcctttgctcggaagagtatgaagatgaacaaagccctgaaaagattatcgagctgtatgcggagtgcatcaggctctttcactccatcgacatatcggattgtccctatacgaatagcttagacagccgcttagccgaattggattacttactgaataacgatctggccgatgtggattgcgaaaactgggaagaagacactccatttaaagatccgcgcgagctgtatgattttttaaagacggaaaagcccgaagaggaacttgtcttttcccacggcgacctgggagacagcaacatctttgtgaaagatggcaaagtaagtggctttattgatcttgggagaagcggcagggcggacaagtggtatgacattgccttctgcgtccggtcgatcagggaggatatcggggaagaacagtatgtcgagctattttttgacttactggggatcaagcctgattgggagaaaataaaatattatattttactggatgaattgttttagtgactgcagtgagatctggtaatgactctctagcttgaggcatcaaataaaacgaaaggctcagtcgaaagactgggcctttcgttttatctgttgtttgtcggtgaacgctctcctgagtaggacaaatccgccgctctagctaagcagaaggccatcctgacggatggcctttttgcgtttctacaaactcttgttaactctagagctgcctgccgcgtttcggtgatgaagatcttcccgatgattaattaattcagaacgctcggttgccgccgggcgttttttatgaagcttcgttgctggcgtttttccataggctccgcccccctgacgagcatcacaaaaatcgacgctcaagtcagaggtggcgaaacccgacaggactataaagataccaggcgtttccccctggaagctccctcgtgcgctctcctgttccgaccctgccgcttaccggatacctgtccgcctttctcccttcgggaagcgtggcgctttctcatagctcacgctgtaggtatctcagttcggtgtaggtcgttcgctccaagctgggctgtgtgcacgaaccccccgttcagcccgaccgctgcgccttatccggtaactatcgtcttgagtccaacccggtaagacacgacttatcgccactggcagcagccactggtaacaggattagcagagcgaggtatgtaggcggtgctacagagttcttgaagtggtggcctaactacggctacactagaaggacagtatttggtatctgcgctctgctgaagccagttaccttcggaaaaagagttggtagctcttgatccggcaaacaaaccaccgctggtagcggtggtttttttgtttgcaagcagcagattacgcgcagaaaaaaaggatctcaagaagatcctttgatcttttctacggggtctgacgctcagtggaacgaaaactcacgttaagggattttggtcatgagattatcaaaaaggatcttcacctagatccttttaaattaaaaatgaagttttaaatcaatctaaagtatatatgagtaaacttggtctgaca

SEQ ID NO: 22 - DNA, 846 bp, Bacillus licheniformis
gtgaacagatcctttaccgttgaaaaggtactcaacaacaacgttttaatcgctctccatgatgattacagagaagttgtcttgattggcaaaggaatcggttttggtaaaaagcgcggagatcttatcgaacatgagaactacgaaaaaatgtttatcctggaaaatgataaggaacaatcgcagtataagaagctcctcacttatgtcgatgaaaaaatggttgatatcgccaatgatgtcatctaccatatcgcgcaaaaaatcggccagccgctgaacgaacacattcatgtcgccctgacggaccatatcgcatttgcagttaagcgtctagaaaagggatttgatatgaaaaatccgtttttgcttgagacggaatcgctttatccgaaggaatacgaagtcgccaaggaagccgtcgatatgattaatgaaaaatccgacattcagctgcctgaaggtgaaatcgggttcatcgcgcttcatatccacagtgcgatgacaaaccgcccgctttctgaagtcaatcagcattcacaactgatctccaggcttgtccaggtcatcgaagattcattccagatgcaagtcaacagggaaagcgtgaactatttgcggctgatcaggcacttgcgctttacgattgacaggataaaacgggacgagccgattcaggaaccggaaaaattaatgttgttgttgaaaacggaatatccgctgtgttacaatactgcttggaagatgatcaagatcttgcagcaagcgctcaagaaaccggttcatgaggcagaagccgtttatttgacattgcatttgtaccgtttgactaataaaatttcataa

SEQ ID NO: 23 - DNA, 23 bp, Bacillus licheniformis
ttttttcatcgacataagtgagg

SEQ ID NO: 24 - DNA, 20 bp, Artificial Sequence
  glcT VT domain
ttttttcatcgacataagtg

SEQ ID NO: 25 - DNA, 3 bp, Artificial Sequence
  glcT target site PAM sequence
agg

SEQ ID NO: 26 - DNA, 76 bp, Artificial Sequence
  Cas9 endonuclease recognition domain
gttttagagctagaaatagcaagttaaaataaggctagtccgttatcaacttgaaaaagtggcaccgagtcggtgc

SEQ ID NO: 27 - RNA, 96 nt, Artificial Sequence
  glcT RNA
uuuuuucaucgacauaagugguuuuagagcuagaaauagcaaguuaaaauaaggcuaguccguuaucaacuugaaaaaguggcaccgagucggugc

SEQ ID NO: 28 - DNA, 96 bp, Artificial Sequence
  DNA encoding glcT gRNA
ttttttcatcgacataagtggttttagagctagaaatagcaagttaaaataaggctagtccgttatcaacttgaaaaagtggcaccgagtcggtgc

SEQ ID NO: 29 - DNA, 93 bp, Bacillus subtilis
tcgctgataaacagctgacatcaactaaaagcttcattaaatactttgaaaaaagttgttgacttaaaagaagctaaatgttatagtaataaa

SEQ ID NO: 30 - DNA, 95 bp, lambda phage
gactcctgttgatagatccagtaatgacctcagaactccatctggatttgttcagaacgctcggttgccgccgggcgttttttattggtgagaat

SEQ ID NO: 31 - DNA, 284 bp, Artificial Sequence
  glcT gRNA expression cassette
tcgctgataaacagctgacatcaactaaaagcttcattaaatactttgaaaaaagttgttgacttaaaagaagctaaatgttatagtaataaattttttcatcgacataagtggttttagagctagaaatagcaagttaaaataaggctagtccgttatcaacttgaaaaagtggcaccgagtcggtgcgactcctgttgatagatccagtaatgacctcagaactccatctggatttgttcagaacgctcggttgccgccgggcgttttttattggtgagaat

SEQ ID NO: 32 - DNA, 500 bp, Bacillus licheniformis
taagctgtgacaaccagccgatcagcgaagtgctcggcatttcaacaattgaaatcaatataaaggaaatggggaagcgcgcgtttcgccttctgcaaaaaagaatcggcggcgccgggccggaaaaactgactgttccttacaagctgatcaaaagggcgactgtgtaatcaaaacatcaatctttttccagacagtgatcaaaattcgacatttttcatcaaaaacgtcaaaataaattgacgcgctttcatgagttttgtacgatatgagagattgatgacaaaaaggagctgaggatcgtgaacagatcctttaccgttgaaaaggtactcaacaacaacgttttaatcgctctccatgatgattacagagaagttgtcttgattggcaaaggaatcggttttggtaaaaagcgcggagatcttatcgaacatgagaactacgaaaaaatgtttatcctggaaaatgataaggaacaatcgcagtataagaagctc

SEQ ID NO: 33 - DNA, 38 bp, Artificial Sequence
  glcT 5' forward primer
tgagtaaacttggtctgacataagctgtgacaaccagc

SEQ ID NO: 34 - DNA, 45 bp, Artificial Sequence
  glcT 5' reverse primer
ccattttttcatcgacataagtgaagagcttcttatactgcgatt

SEQ ID NO: 35 - DNA, 500 bp, Bacillus licheniformis
tcacttatgtcgatgaaaaaatggttgatatcgccaatgatgtcatctaccatatcgcgcaaaaaatcggccagccgctgaacgaacacattcatgtcgccctgacggaccatatcgcatttgcagttaagcgtctagaaaagggatttgatatgaaaaatccgtttttgcttgagacggaatcgctttatccgaaggaatacgaagtcgccaaggaagccgtcgatatgattaatgaaaaatccgacattcagctgcctgaaggtgaaatcgggttcatcgcgcttcatatccacagtgcgatgacaaaccgcccgctttctgaagtcaatcagcattcacaactgatctccaggcttgtccaggtcatcgaagattcattccagatgcaagtcaacagggaaagcgtgaactatttgcggctgatcaggcacttgcgctttacgattgacaggataaaacgggacgagccgattcaggaaccggaaaaattaatgttg

SEQ ID NO: 36 - DNA, 45 bp, Artificial Sequence
  glcT 3' forward primer
aatcgcagtataagaagctcttcacttatgtcgatgaaaaaatgg

SEQ ID NO: 37 - DNA, 46 bp, Artificial Sequence
  glcT 3' reverse primer
cagaagaaaatggaggaattccaacattaatttttccggttcctga

SEQ ID NO: 38 - DNA, 9632 bp, Artificial Sequence
  pRF731
tcgctgataaacagctgacatcaactaaaagcttcattaaatactttgaaaaaagttgttgacttaaaagaagctaaatgttatagtaataaattttttcatcgacataagtggttttagagctagaaatagcaagttaaaataaggctagtccgttatcaacttgaaaaagtggcaccgagtcggtgcgactcctgttgatagatccagtaatgacctcagaactccatctggatttgttcagaacgctcggttgccgccgggcgttttttattggtgagaatgaattcgcggccgcacgcgtccatggggatccccgcgggtcgacctcgagagttacgctagggataacagggtaatataggagctccagtcggcttaaaccagttttcgctggtgcgaaaaaagagtgtcttgtgacacctaaattcaaaatctatcggtcagatttataccgatttgattttatatattcttgaataacatacgccgagttatcacataaaagcgggaaccaatcataaaatttaaacttcattgcataatccattaaactcttaaattctacgattccttgttcatcaataaactcaatcatttctttaattaatttatatctatctgttgttgttttctttaataattcattaacatctacaccgccataaactatcatatcttctttttgatatttaaatttattaggatcgtccatgtgaagcatatatctcacaagacctttcacacttcctgcaatctgcggaatagtcgcattcaattcttctgttaattatttttatctgttcataagatttattaccctcatacatcactagaatatgataatgctcttttttcatcctaccttctgtatcagtatccctatcatgtaatggagacactacaaattgaatgtgtaactcttttaaatactctaaccactcggcttttgctgattctggatataaaacaaatgtccaattacgtcctcttgaatttttcttgttttcagtttcttttattacattttcgctcatgatataataacggtgctaatacacttaacaaaatttagtcatagataggcagcatgccagtgctgtctatctttttttgtttaaaatgcaccgtattcctcctttgcatatttttttattagaataccggttgcatctgatttgctaatattatatttttctttgattctatttaatatctcattttcttctgttgtaagtcttaaagtaacagcaacttttttctcttcttttctatctacaactatcactgtacctcccaacatctgtttttttcactttaacataaaaaacaaccttttaacattaaaaacccaatatttatttatttgtttggacaatggacactggacacctaggggggaggtcgtagtacccccctatgttttctcccctaaataaccccaaaaatctaagaaaaaaagacctcaaaaaggtctttaattaacatctcaaatttcgcatttattccaatttcctttttgcgtgtgatgcgagctcatcggctccgtcgatactatgttatacgccaactttcaaaacaactttgaaaaagctgttttctggtatttaaggttttagaatgcaaggaacagtgaattggagttcgtcttgttataattagcttcttggggtatctttaaatactgtagaaaagaggaaggaaataataaatggctaaaatgagaatatcaccggaattgaaaaaactgatcgaaaaataccgctgcgtaaaagatacggaaggaatgtctcctgctaaggtatataagctggtgggagaaaatgaaaacctatatttaaaaatgacggacagccggtataaagggaccacctatgatgtggaacgggaaaaggacatgatgctatggctggaaggaaagctgcctgttccaaaggtcctgcactttgaacggcatgatggctggagcaatctgctcatgagtgaggccgatggcgtcctttgctcggaagagtatgaagatgaacaaagccctgaaaagattatcgagctgtatgcggagtgcatcaggctctttcactccatcgacatatcggattgtccctatacgaatagcttagacagccgcttagccgaattggattacttactgaataacgatctggccgatgtggattgcgaaaactgggaagaagacactccatttaaagatccgcgcgagctgtatgattttttaaagacggaaaagcccgaagaggaacttgtcttttcccacggcgacctgggagacagcaacatctttgtgaaagatggcaaagtaagtggctttattgatcttgggagaagcggcagggcggacaagtggtatgacattgccttctgcgtccggtcgatcagggaggatatcggggaagaacagtatgtcgagctattttttgacttactggggatcaagcctgattgggagaaaataaaatattatattttactggatgaattgttttagtgactgcagtgagatctggtaatgactctctagcttgaggcatcaaataaaacgaaaggctcagtcgaaagactgggcctttcgttttatctgttgtttgtcggtgaacgctctcctgagtaggacaaatccgccgctctagctaagcagaaggccatcctgacggatggcctttttgcgtttctacaaactcttgttaactctagagctgcctgccgcgtttcggtgatgaagatcttcccgatgattaattaattcagaacgctcggttgccgccgggcgttttttatgaagcttcgttgctggcgtttttccataggctccgcccccctgacgagcatcacaaaaatcgacgctcaagtcagaggtggcgaaacccgacaggactataaagataccaggcgtttccccctggaagctccctcgtgcgctctcctgttccgaccctgccgcttaccggatacctgtccgcctttctcccttcgggaagcgtggcgctttctcatagctcacgctgtaggtatctcagttcggtgtaggtcgttcgctccaagctgggctgtgtgcacgaaccccccgttcagcccgaccgctgcgccttatccggtaactatcgtcttgagtccaacccggtaagacacgacttatcgccactggcagcagccactggtaacaggattagcagagcgaggtatgtaggcggtgctacagagttcttgaagtggtggcctaactacggctacactagaaggacagtatttggtatctgcgctctgctgaagccagttaccttcggaaaaagagttggtagctcttgatccggcaaacaaaccaccgctggtagcggtggtttttttgtttgcaagcagcagattacgcgcagaaaaaaaggatctcaagaagatcctttgatcttttctacggggtctgacgctcagtggaacgaaaactcacgttaagggattttggtcatgagattatcaaaaaggatcttcacctagatccttttaaattaaaaatgaagttttaaatcaatctaaagtatatatgagtaaacttggtctgacataagctgtgacaaccagccgatcagcgaagtgctcggcatttcaacaattgaaatcaatataaaggaaatggggaagcgcgcgtttcgccttctgcaaaaaagaatcggcggcgccgggccggaaaaactgactgttccttacaagctgatcaaaagggcgactgtgtaatcaaaacatcaatctttttccagacagtgatcaaaattcgacatttttcatcaaaaacgtcaaaataaattgacgcgctttcatgagttttgtacgatatgagagattgatgacaaaaaggagctgaggatcgtgaacagatcctttaccgttgaaaaggtactcaacaacaacgttttaatcgctctccatgatgattacagagaagttgtcttgattggcaaaggaatcggttttggtaaaaagcgcggagatcttatcgaacatgagaactacgaaaaaatgtttatcctggaaaatgataaggaacaatcgcagtataagaagctcttcacttatgtcgatgaaaaaatggttgatatcgccaatgatgtcatctaccatatcgcgcaaaaaatcggccagccgctgaacgaacacattcatgtcgccctgacggaccatatcgcatttgcagttaagcgtctagaaaagggatttgatatgaaaaatccgtttttgcttgagacggaatcgctttatccgaaggaatacgaagtcgccaaggaagccgtcgatatgattaatgaaaaatccgacattcagctgcctgaaggtgaaatcgggttcatcgcgcttcatatccacagtgcgatgacaaaccgcccgctttctgaagtcaatcagcattcacaactgatctccaggcttgtccaggtcatcgaagattcattccagatgcaagtcaacagggaaagcgtgaactatttgcggctgatcaggcacttgcgctttacgattgacaggataaaacgggacgagccgattcaggaaccggaaaaattaatgttggaattcctccattttcttctgctatcaaaataacagactcgtgattttccaaacgagctttcaaaaaagcctctgccccttgcaaatcggatgcctgtctataaaattcccgatattggttaaacagcggcgcaatggcggccgcatctgatgtctttgcttggcgaatgttcatcttatttcttcctccctctcaataattttttcattctatcccttttctgtaaagtttatttttcagaatacttttatcatcatgctttgaaaaaatatcacgataatatccattgttctcacggaagcacacgcaggtcatttgaacgaattttttcgacaggaatttgccgggactcaggagcatttaacctaaaaaagcatgacatttcagcataatgaacatttactcatgtctattttcgttcttttctgtatgaaaatagttatttcgagtctctacggaaatagcgagagatgatatacctaaatagagataaaatcatctcaaaaaaatgggtctactaaaatattattccatctattacaataaattcacagaatagtcttttaagtaagtctactctgaatttttttaaaaggagagggtaactagtggccccaaaaaagaaacgcaaggttatggataaaaaatacagcattggtctggatatcggaaccaacagcgttgggtgggcagtaataacagatgaatacaaagtgccgtcaaaaaaatttaaggttctggggaatacagatcgccacagcataaaaaagaatctgattggggcattgctgtttgattcgggtgagacagctgaggccacgcgtctgaaacgtacagcaagaagacgttacacacgtcgtaaaaatcgtatttgctacttacaggaaattttttctaacgaaatggccaaggtagatgatagtttcttccatcgtctcgaagaatcttttctggttgaggaagataaaaaacacgaacgtcaccctatctttggcaatatcgtggatgaagtggcctatcatgaaaaataccctacgatttatcatcttcgcaagaagttggttgatagtacggacaaagcggatctgcgtttaatctatcttgcgttagcgcacatgatcaaatttcgtggtcatttcttaattgaaggtgatctgaatcctgataactctgatgtggacaaattgtttatacaattagtgcaaacctataatcagctgttcgaggaaaaccccattaatgcctctggagttgatgccaaagcgattttaagcgcgagactttctaagtcccggcgtctggagaatctgatcgcccagttaccaggggaaaagaaaaatggtctgtttggtaatctgattgccctcagtctggggcttaccccgaacttcaaatccaattttgacctggctgaggacgcaaagctgcagctgagcaaagatacttatgatgatgacctcgacaatctgctcgcccagattggtgaccaatatgcggatctgtttctggcagcgaagaatctttcggatgctatcttgctgtcggatattctgcgtgttaataccgaaatcaccaaagcgcctctgtctgcaagtatgatcaagagatacgacgagcaccaccaggacctgactcttcttaaggcactggtacgccaacagcttccggagaaatacaaagaaatattcttcgaccagtccaagaatggttacgcgggctacatcgatggtggtgcatcacaggaagagttctataaatttattaaaccaatccttgagaaaatggatggcacggaagagttacttgttaaacttaaccgcgaagacttgcttagaaagcaacgtacattcgacaacggctccatcccacaccagattcatttaggtgaacttcacgccatcttgcgcagacaagaagatttctatcccttcttaaaagacaatcgggagaaaatcgagaagatcctgacgttccgcattccctattatgtcggtcccctggcacgtggtaattctcggtttgcctggatgacgcgcaaaagtgaggaaaccatcaccccttggaactttgaagaagtcgtggataaaggtgctagcgcgcagtcttttatagaaagaatgacgaacttcgataaaaacttgcccaacgaaaaagtcctgcccaagcactctcttttatatgagtactttactgtgtacaacgaactgactaaagtgaaatacgttacggaaggtatgcgcaaacctgcctttcttagtggcgagcagaaaaaagcaattgtcgatcttctctttaaaacgaatcgcaaggtaactgtaaaacagctgaaggaagattatttcaaaaagatcgaatgctttgattctgtcgagatctcgggtgtcgaagatcgtttcaacgcttccttagggacctatcatgatttgctgaagataataaaagacaaagactttctcgacaatgaagaaaatgaagatattctggaggatattgttttgaccttgaccttattcgaagatagagagatgatcgaggagcgcttaaaaacctatgcccacctgtttgatgacaaagtcatgaagcaattaaagcgccgcagatatacggggtggggccgcttgagccgcaagttgattaacggtattagagacaagcagagcggaaaaactatcctggatttcctcaaatctgacggatttgcgaaccgcaattttatgcagcttatacatgatgattcgcttacattcaaagaggatattcagaaggctcaggtgtctgggcaaggtgattcactccacgaacatatagcaaatttggccggctctcctgcgattaagaaggggatcctgcaaacagttaaagttgtggatgaacttgtaaaagtaatgggccgccacaagccggagaatatcgtgatagaaatggcgcgcgagaatcaaacgacacaaaaaggtcaaaagaactcaagagagagaatgaagcgcattgaggaggggataaaggaacttggatctcaaattctgaaagaacatccagttgaaaacactcagctgcaaaatgaaaaattgtacctgtactacctgcagaatggaagagacatgtacgtggatcaggaattggatatcaatagactctcggactatgacgtagatcacattgtccctcagagcttcctcaaggatgattctatagataataaagtacttacgagatcggacaaaaatcgcggtaaatcggataacgtcccatcggaggaagtcgttaaaaagatgaaaaactattggcgtcaactgctgaacgccaagctgatcacacagcgtaagtttgataatctgactaaagccgaacgcggtggtcttagtgaactcgataaagcaggatttataaaacggcagttagtagaaacgcgccaaattacgaaacacgtggctcagatcctcgattctagaatgaatacaaagtacgatgaaaacgataaactgatccgtgaagtaaaagtcattaccttaaaatctaaacttgtgtccgatttccgcaaagattttcagttttacaaggtccgggaaatcaataactatcaccatgcacatgatgcatatttaaatgcggttgtaggcacggcccttattaagaaataccctaaactcgaaagtgagtttgtttatggggattataaagtgtatgacgttcgcaaaatgatcgcgaaatcagaacaggaaatcggtaaggctaccgctaaatactttttttattccaacattatgaatttttttaagaccgaaataactctcgcgaatggtgaaatccgtaaacggcctcttatagaaaccaatggtgaaacgggagaaatcgtttgggataaaggtcgtgactttgccaccgttcgtaaagtcctctcaatgccgcaagttaacattgtcaagaagacggaagttcaaacagggggattctccaaagaatctatcctgccgaagcgtaacagtgataaacttattgccagaaaaaaagattgggatccaaaaaaatacggaggctttgattcccctaccgtcgcgtatagtgtgctggtggttgctaaagtcgagaaagggaaaagcaagaaattgaaatcagttaaagaactgctgggtattacaattatggaaagatcgtcctttgagaaaaatccgatcgactttttagaggccaaggggtataaggaagtgaaaaaagatctcatcatcaaattaccgaagtatagtctttttgagctggaaaacggcagaaaaagaatgctggcctccgcgggcgagttacagaagggaaatgagctggcgctgccttccaaatatgttaattttctgtaccttgccagtcattatgagaaactgaagggcagccccgaagataacgaacagaaacaattattcgtggaacagcataagcactatttagatgaaattatagagcaaattagtgaattttctaagcgcgttatcctcgcggatgctaatttagacaaagtactgtcagcttataataaacatcgggataagccgattagagaacaggccgaaaatatcattcatttgtttaccttaaccaaccttggagcaccagctgccttcaaatatttcgataccacaattgatcgtaaacggtatacaagtacaaaagaagtcttggacgcaaccctcattcatcaatctattactggattatatgagacacgcattgatctttcacagctgggcggagacaagaagaaaaaactgaaactgcaccatcatcaccatcatcatcaccatcattgataactcgagaaagcttacataaaaaaccggccttggccccgccggttttttattatttttcttcctccgcatgttcaatccgctccataatcgacggatggctccctctgaaaattttaacgagaaacggcgggttgacccggctcagtcccgtaacggccaagtcctgaaacgtctcaatcgccgcttcccggtttccggtcagctcaatgccgtaacggtcggcggcgttttcctgataccgggagacggcattcgtaatc

SEQ ID NO: 39 - DNA, 9632 bp, Artificial Sequence
  pRF724
gaattcctccattttcttctgctatcaaaataacagactcgtgattttccaaacgagctttcaaaaaagcctctgccccttgcaaatcggatgcctgtctataaaattcccgatattggttaaacagcggcgcaatggcggccgcatctgatgtctttgcttggcgaatgttcatcttatttcttcctccctctcaataattttttcattctatcccttttctgtaaagtttatttttcagaatacttttatcatcatgctttgaaaaaatatcacgataatatccattgttctcacggaagcacacgcaggtcatttgaacgaattttttcgacaggaatttgccgggactcaggagcatttaacctaaaaaagcatgacatttcagcataatgaacatttactcatgtctattttcgttcttttctgtatgaaaatagttatttcgagtctctacggaaatagcgagagatgatatacctaaatagagataaaatcatctcaaaaaaatgggtctactaaaatattattccatctattacaataaattcacagaatagtcttttaagtaagtctactctgaatttttttaaaaggagagggtaactagtggccccaaaaaagaaacgcaaggttatggataaaaaatacagcattggtctggatatcggaaccaacagcgttgggtgggcagtaataacagatgaatacaaagtgccgtcaaaaaaatttaaggttctggggaatacagatcgccacagcataaaaaagaatctgattggggcattgctgtttgattcgggtgagacagctgaggccacgcgtctgaaacgtacagcaagaagacgttacacacgtcgtaaaaatcgtatttgctacttacaggaaattttttctaacgaaatggccaaggtagatgatagtttcttccatcgtctcgaagaatcttttctggttgaggaagataaaaaacacgaacgtcaccctatctttggcaatatcgtggatgaagtggcctatcatgaaaaataccctacgatttatcatcttcgcaagaagttggttgatagtacggacaaagcggatctgcgtttaatctatcttgcgttagcgcacatgatcaaatttcgtggtcatttcttaattgaaggtgatctgaatcctgataactctgatgtggacaaattgtttatacaattagtgcaaacctataatcagctgttcgaggaaaaccccattaatgcctctggagttgatgccaaagcgattttaagcgcgagactttctaagtcccggcgtctggagaatctgatcgcccagttaccaggggaaaagaaaaatggtctgtttggtaatctgattgccctcagtctggggcttaccccgaacttcaaatccaattttgacctggctgaggacgcaaagctgcagctgagcaaagatacttatgatgatgacctcgacaatctgctcgcccagattggtgaccaatatgcggatctgtttctggcagcgaagaatctttcggatgctatcttgctgtcggatattctgcgtgttaataccgaaatcaccaaagcgcctctgtctgcaagtatgatcaagagatacgacgagcaccaccaggacctgactcttcttaaggcactggtacgccaacagcttccggagaaatacaaagaaatattcttcgaccagtccaagaatggttacgcgggctacatcgatggtggtgcatcacaggaagagttctataaatttattaaaccaatccttgagaaaatggatggcacggaagagttacttgttaaacttaaccgcgaagacttgcttagaaagcaacgtacattcgacaacggctccatcccacaccagattcatttaggtgaacttcacgccatcttgcgcagacaagaagatttctatcccttcttaaaagacaatcgggagaaaatcgagaagatcctgacgttccgcattccctattatgtcggtcccctggcacgtggtaattctcggtttgcctggatgacgcgcaaaagtgaggaaaccatcaccccttggaactttgaagaagtcgtggataaaggtgctagcgcgcagtcttttatagaaagaatgacgaacttcgataaaaacttgcccaacgaaaaagtcctgcccaagcactctcttttatatgagtactttactgtgtacaacgaactgactaaagtgaaatacgttacggaaggtatgcgcaaacctgcctttcttagtggcgagcagaaaaaagcaattgtcgatcttctctttaaaacgaatcgcaaggtaactgtaaaacagctgaaggaagattatttcaaaaagatcgaatgctttgattctgtcgagatctcgggtgtcgaagatcgtttcaacgcttccttagggacctatcatgatttgctgaagataataaaagacaaagactttctcgacaatgaagaaaatgaagatattctggaggatattgttttgaccttgaccttattcgaagatagagagatgatcgaggagcgcttaaaaacctatgcccacctgtttgatgacaaagtcatgaagcaattaaagcgccgcagatatacggggtggggccgcttgagccgcaagttgattaacggtattagagacaagcagagcggaaaaactatcctggatttcctcaaatctgacggatttgcgaaccgcaattttatgcagcttatacatgatgattcgcttacattcaaagaggatattcagaaggctcaggtgtctgggcaaggtgattcactccacgaacatatagcaaatttggccggctctcctgcgattaagaaggggatcctgcaaacagttaaagttgtggatgaacttgtaaaagtaatgggccgccacaagccggagaatatcgtgatagaaatggcgcgcgagaatcaaacgacacaaaaaggtcaaaagaactcaagagagagaatgaagcgcattgaggaggggataaaggaacttggatctcaaattctgaaagaacatccagttgaaaacactcagctgcaaaatgaaaaattgtacctgtactacctgcagaatggaagagacatgtacgtggatcaggaattggatatcaatagactctcggactatgacgtagatcacattgtccctcagagcttcctcaaggatgattctatagataataaagtacttacgagatcggacaaaaatcgcggtaaatcggataacgtcccatcggaggaagtcgttaaaaagatgaaaaactattggcgtcaactgctgaacgccaagctgatcacacagcgtaagtttgataatctgactaaagccgaacgcggtggtcttagtgaactcgataaagcaggatttataaaacggcagttagtagaaacgcgccaaattacgaaacacgtggctcagatcctcgattctagaatgaatacaaagtacgatgaaaacgataaactgatccgtgaagtaaaagtcattaccttaaaatctaaacttgtgtccgatttccgcaaagattttcagttttacaaggtccgggaaatcaataactatcaccatgcacatgatgcatatttaaatgcggttgtaggcacggcccttattaagaaataccctaaactcgaaagtgagtttgtttatggggattataaagtgtatgacgttcgcaaaatgatcgcgaaatcagaacaggaaatcggtaaggctaccgctaaatactttttttattccaacattatgaatttttttaagaccgaaataactctcgcgaatggtgaaatccgtaaacggcctcttatagaaaccaatggtgaaacgggagaaatcgtttgggataaaggtcgtgactttgccaccgttcgtaaagtcctctcaatgccgcaagttaacattgtcaagaagacggaagttcaaacagggggattctccaaagaatctatcctgccgaagcgtaacagtgataaacttattgccagaaaaaaagattgggatccaaaaaaatacggaggctttgattcccctaccgtcgcgtatagtgtgctggtggttgctaaagtcgagaaagggaaaagcaagaaattgaaatcagttaaagaactgctgggtattacaattatggaaagatcgtcctttgagaaaaatccgatcgactttttagaggccaaggggtataaggaagtgaaaaaagatctcatcatcaaattaccgaagtatagtctttttgagctggaaaacggcagaaaaagaatgctggcctccgcgggcgagttacagaagggaaatgagctggcgctgccttccaaatatgttaattttctgtaccttgccagtcattatgagaaactgaagggcagccccgaagataacgaacagaaacaattattcgtggaacagcataagcactatttagatgaaattatagagcaaattagtgaattttctaagcgcgttatcctcgcggatgctaatttagacaaagtactgtcagcttataataaacatcgggataagccgattagagaacaggccgaaaatatcattcatttgtttaccttaaccaaccttggagcaccagctgccttcaaatatttcgataccacaattgatcgtaaacggtatacaagtacaaaagaagtcttggacgcaaccctcattcatcaatctattactggattatatgagacacgcattgatctttcacagctgggcggagacaagaagaaaaaactgaaactgcaccatcatcaccatcatcatcaccatcattgataactcgagaaagcttacataaaaaaccggccttggccccgccggttttttattatttttcttcctccgcatgttcaatccgctccataatcgacggatggctccctctgaaaattttaacgagaaacggcgggttgacccggctcagtcccgtaacggccaagtcctgaaacgtctcaatcgccgcttcccggtttccggtcagctcaatgccgtaacggtcggcggcgttttcctgataccgggagacggcattcgtaatcgtatgaggaactgatggcatctgcaggctatatcagcgcgtctacagtccaggaagcaagaagcagctatgattccatttacgacatcgtgtcacagtacgatttagaggacctttctctgtttgacagcgaaaagtggaaggtgctttcaaaaaaagacatcgaaaacctggacaaatatttcgactttctcgtgcaggaagcaagcagccgaaacaaaaactgaatacttctccgcggcacactctcctctctatcattttcgtctgtttacgatcctgctgttattttatcccttatgttaacttttgtcaatatttttcctgtctaagtatttcctatagtcaacatttgtattaaaatgttcatatcatgaatttgcgggggggatggcgatgacaaggttcggcgagcggctcaaagagctgagggaacaaagaagcctgtcggttaatcagcttgccatgtatgccggtgtgagcgccgcagccatttccagaatcgaaaacggccaccgcggcgttcccaagcccgcgacgatcagaaaattggccgaggctctgaaaatgccgtacgagcagctcatggatattgccggttatatgagagctgacgagattcgcgaacagccgcgcggctatgtcacgatgcaggagatcgcggccaagcacggcgtcgaagacctgtggctgtttaaacccgagaaatgggactgtttgtcccgcgaagacctgctcaacctcgaacagtattttcattttttggttaatgaagcgaagaagcgccaatcataaaaagccgaatttcccttttaggagaagttcggcttttttcggctgccttaagcggcatccggattcggcgtcttgcctttatgatgcttaacggggctcagcgcacgctcgagccatcccatgaacagatcggcgatgatcgccatcagcgccgtcgggatcgcgcctgctagaatgatcgctgttccgttggtcgcgtttgatcctcgctgataaacagctgacatcaactaaaagcttcattaaatactttgaaaaaagttgttgacttaaaagaagctaaatgttatagtaataaaaaatggctgcggctctggaaagttttagagctagaaatagcaagttaaaataaggctagtccgttatcaacttgaaaaagtggcaccgagtcggtgcgactcctgttgatagatccagtaatgacctcagaactccatctggatttgttcagaacgctcggttgccgccgggcgttttttattggtgagaatgaattcgcggccgcacgcgtccatggggatccccgcgggtcgacctcgagagttacgctagggataacagggtaatataggagctccagtcggcttaaaccagttttcgctggtgcgaaaaaagagtgtcttgtgacacctaaattcaaaatctatcggtcagatttataccgatttgattttatatattcttgaataacatacgccgagttatcacataaaagcgggaaccaatcataaaatttaaacttcattgcataatccattaaactcttaaattctacgattccttgttcatcaataaactcaatcatttctttaattaatttatatctatctgttgttgttttctttaataattcattaacatctacaccgccataaactatcatatcttctttttgatatttaaatttattaggatcgtccatgtgaagcatatatctcacaagacctttcacacttcctgcaatctgcggaatagtcgcattcaattcttctgttaattatttttatctgttcataagatttattaccctcatacatcactagaatatgataatgctcttttttcatcctaccttctgtatcagtatccctatcatgtaatggagacactacaaattgaatgtgtaactcttttaaatactctaaccactcggcttttgctgattctggatataaaacaaatgtccaattacgtcctcttgaatttttcttgttttcagtttcttttattacattttcgctcatgatataataacggtgctaatacacttaacaaaatttagtcatagataggcagcatgccagtgctgtctatctttttttgtttaaaatgcaccgtattcctcctttgcatatttttttattagaataccggttgcatctgatttgctaatattatatttttctttgattctatttaatatctcattttcttctgttgtaagtcttaaagtaacagcaacttttttctcttcttttctatctacaactatcactgtacctcccaacatctgtttttttcactttaacataaaaaacaaccttttaacattaaaaacccaatatttatttatttgtttggacaatggacactggacacctaggggggaggtcgtagtacccccctatgttttctcccctaaataaccccaaaaatctaagaaaaaaagacctcaaaaaggtctttaattaacatctcaaatttcgcatttattccaatttcctttttgcgtgtgatgcgagctcatcggctccgtcgatactatgttatacgccaactttcaaaacaactttgaaaaagctgttttctggtatttaaggttttagaatgcaaggaacagtgaattggagttcgtcttgttataattagcttcttggggtatctttaaatactgtagaaaagaggaaggaaataataaatggctaaaatgagaatatcaccggaattgaaaaaactgatcgaaaaataccgctgcgtaaaagatacggaaggaatgtctcctgctaaggtatataagctggtgggagaaaatgaaaacctatatttaaaaatgacggacagccggtataaagggaccacctatgatgtggaacgggaaaaggacatgatgctatggctggaaggaaagctgcctgttccaaaggtcctgcactttgaacggcatgatggctggagcaatctgctcatgagtgaggccgatggcgtcctttgctcggaagagtatgaagatgaacaaagccctgaaaagattatcgagctgtatgcggagtgcatcaggctctttcactccatcgacatatcggattgtccctatacgaatagcttagacagccgcttagccgaattggattacttactgaataacgatctggccgatgtggattgcgaaaactgggaagaagacactccatttaaagatccgcgcgagctgtatgattttttaaagacggaaaagcccgaagaggaacttgtcttttcccacggcgacctgggagacagcaacatctttgtgaaagatggcaaagtaagtggctttattgatcttgggagaagcggcagggcggacaagtggtatgacattgccttctgcgtccggtcgatcagggaggatatcggggaagaacagtatgtcgagctattttttgacttactggggatcaagcctgattgggagaaaataaaatattatattttactggatgaattgttttagtgactgcagtgagatctggtaatgactctctagcttgaggcatcaaataaaacgaaaggctcagtcgaaagactgggcctttcgttttatctgttgtttgtcggtgaacgctctcctgagtaggacaaatccgccgctctagctaagcagaaggccatcctgacggatggcctttttgcgtttctacaaactcttgttaactctagagctgcctgccgcgtttcggtgatgaagatcttcccgatgattaattaattcagaacgctcggttgccgccgggcgttttttatgaagcttcgttgctggcgtttttccataggctccgcccccctgacgagcatcacaaaaatcgacgctcaagtcagaggtggcgaaacccgacaggactataaagataccaggcgtttccccctggaagctccctcgtgcgctctcctgttccgaccctgccgcttaccggatacctgtccgcctttctcccttcgggaagcgtggcgctttctcatagctcacgctgtaggtatctcagttcggtgtaggtcgttcgctccaagctgggctgtgtgcacgaaccccccgttcagcccgaccgctgcgccttatccggtaactatcgtcttgagtccaacccggtaagacacgacttatcgccactggcagcagccactggtaacaggattagcagagcgaggtatgtaggcggtgctacagagttcttgaagtggtggcctaactacggctacactagaaggacagtatttggtatctgcgctctgctgaagccagttaccttcggaaaaagagttggtagctcttgatccggcaaacaaaccaccgctggtagcggtggtttttttgtttgcaagcagcagattacgcgcagaaaaaaaggatctcaagaagatcctttgatcttttctacggggtctgacgctcagtggaacgaaaactcacgttaagggattttggtcatgagattatcaaaaaggatcttcacctagatccttttaaattaaaaatgaagttttaaatcaatctaaagtatatatgagtaaacttggtctgaca

SEQ ID NO: 40 - DNA, 18 bp, Bacillus licheniformis
gccgcagccatttccaga

SEQ ID NO: 41 - DNA, 417 bp, Bacillus licheniformis
atgacaaggttcggcgagcggctcaaagagctgagggaacaaagaagcctgtcggttaatcagcttgccatgtatgccggtgtgagcgccgcagccatttccagagccgcagccatttccagaatcgaaaacggccaccgcggcgttcccaagcccgcgacgatcagaaaattggccgaggctctgaaaatgccgtacgagcagctcatggatattgccggttatatgagagctgacgagattcgcgaacagccgcgcggctatgtcacgatgcaggagatcgcggccaagcacggcgtcgaagacctgtggctgtttaaacccgagaaatgggactgtttgtcccgcgaagacctgctcaacctcgaacagtattttcattttttggttaatgaagcgaagaagcgccaatcataa

SEQ ID NO: 42 - DNA, 8347 bp, Artificial Sequence
  8.3kb PCR of pRF694
gaattcgcggccgcacgcgtccatggggatccccgcgggtcgacctcgagagttacgctagggataacagggtaatataggagctccagtcggcttaaaccagttttcgctggtgcgaaaaaagagtgtcttgtgacacctaaattcaaaatctatcggtcagatttataccgatttgattttatatattcttgaataacatacgccgagttatcacataaaagcgggaaccaatcataaaatttaaacttcattgcataatccattaaactcttaaattctacgattccttgttcatcaataaactcaatcatttctttaattaatttatatctatctgttgttgttttctttaataattcattaacatctacaccgccataaactatcatatcttctttttgatatttaaatttattaggatcgtccatgtgaagcatatatctcacaagacctttcacacttcctgcaatctgcggaatagtcgcattcaattcttctgttaattatttttatctgttcataagatttattaccctcatacatcactagaatatgataatgctcttttttcatcctaccttctgtatcagtatccctatcatgtaatggagacactacaaattgaatgtgtaactcttttaaatactctaaccactcggcttttgctgattctggatataaaacaaatgtccaattacgtcctcttgaatttttcttgttttcagtttcttttattacattttcgctcatgatataataacggtgctaatacacttaacaaaatttagtcatagataggcagcatgccagtgctgtctatctttttttgtttaaaatgcaccgtattcctcctttgcatatttttttattagaataccggttgcatctgatttgctaatattatatttttctttgattctatttaatatctcattttcttctgttgtaagtcttaaagtaacagcaacttttttctcttcttttctatctacaactatcactgtacctcccaacatctgtttttttcactttaacataaaaaacaaccttttaacattaaaaacccaatatttatttatttgtttggacaatggacactggacacctaggggggaggtcgtagtacccccctatgttttctcccctaaataaccccaaaaatctaagaaaaaaagacctcaaaaaggtctttaattaacatctcaaatttcgcatttattccaatttcctttttgcgtgtgatgcgagctcatcggctccgtcgatactatgttatacgccaactttcaaaacaactttgaaaaagctgttttctggtatttaaggttttagaatgcaaggaacagtgaattggagttcgtcttgttataattagcttcttggggtatctttaaatactgtagaaaagaggaaggaaataataaatggctaaaatgagaatatcaccggaattgaaaaaactgatcgaaaaataccgctgcgtaaaagatacggaaggaatgtctcctgctaaggtatataagctggtgggagaaaatgaaaacctatatttaaaaatgacggacagccggtataaagggaccacctatgatgtggaacgggaaaaggacatgatgctatggctggaaggaaagctgcctgttccaaaggtcctgcactttgaacggcatgatggctggagcaatctgctcatgagtgaggccgatggcgtcctttgctcggaagagtatgaagatgaacaaagccctgaaaagattatcgagctgtatgcggagtgcatcaggctctttcactccatcgacatatcggattgtccctatacgaatagcttagacagccgcttagccgaattggattacttactgaataacgatctggccgatgtggattgcgaaaactgggaagaagacactccatttaaagatccgcgcgagctgtatgattttttaaagacggaaaagcccgaagaggaacttgtcttttcccacggcgacctgggagacagcaacatctttgtgaaagatggcaaagtaagtggctttattgatcttgggagaagcggcagggcggacaagtggtatgacattgccttctgcgtccggtcgatcagggaggatatcggggaagaacagtatgtcgagctattttttgacttactggggatcaagcctgattgggagaaaataaaatattatattttactggatgaattgttttagtgactgcagtgagatctggtaatgactctctagcttgaggcatcaaataaaacgaaaggctcagtcgaaagactgggcctttcgttttatctgttgtttgtcggtgaacgctctcctgagtaggacaaatccgccgctctagctaagcagaaggccatcctgacggatggcctttttgcgtttctacaaactcttgttaactctagagctgcctgccgcgtttcggtgatgaagatcttcccgatgattaattaattcagaacgctcggttgccgccgggcgttttttatgaagcttcgttgctggcgtttttccataggctccgcccccctgacgagcatcacaaaaatcgacgctcaagtcagaggtggcgaaacccgacaggactataaagataccaggcgtttccccctggaagctccctcgtgcgctctcctgttccgaccctgccgcttaccggatacctgtccgcctttctcccttcgggaagcgtggcgctttctcatagctcacgctgtaggtatctcagttcggtgtaggtcgttcgctccaagctgggctgtgtgcacgaaccccccgttcagcccgaccgctgcgccttatccggtaactatcgtcttgagtccaacccggtaagacacgacttatcgccactggcagcagccactggtaacaggattagcagagcgaggtatgtaggcggtgctacagagttcttgaagtggtggcctaactacggctacactagaaggacagtatttggtatctgcgctctgctgaagccagttaccttcggaaaaagagttggtagctcttgatccggcaaacaaaccaccgctggtagcggtggtttttttgtttgcaagcagcagattacgcgcagaaaaaaaggatctcaagaagatcctttgatcttttctacggggtctgacgctcagtggaacgaaaactcacgttaagggattttggtcatgagattatcaaaaaggatcttcacctagatccttttaaattaaaaatgaagttttaaatcaatctaaagtatatatgagtaaacttggtctgacagaattcctccattttcttctgctatcaaaataacagactcgtgattttccaaacgagctttcaaaaaagcctctgccccttgcaaatcggatgcctgtctataaaattcccgatattggttaaacagcggcgcaatggcggccgcatctgatgtctttgcttggcgaatgttcatcttatttcttcctccctctcaataattttttcattctatcccttttctgtaaagtttatttttcagaatacttttatcatcatgctttgaaaaaatatcacgataatatccattgttctcacggaagcacacgcaggtcatttgaacgaattttttcgacaggaatttgccgggactcaggagcatttaacctaaaaaagcatgacatttcagcataatgaacatttactcatgtctattttcgttcttttctgtatgaaaatagttatttcgagtctctacggaaatagcgagagatgatatacctaaatagagataaaatcatctcaaaaaaatgggtctactaaaatattattccatctattacaataaattcacagaatagtcttttaagtaagtctactctgaatttttttaaaaggagagggtaactagtggccccaaaaaagaaacgcaaggttatggataaaaaatacagcattggtctggatatcggaaccaacagcgttgggtgggcagtaataacagatgaatacaaagtgccgtcaaaaaaatttaaggttctggggaatacagatcgccacagcataaaaaagaatctgattggggcattgctgtttgattcgggtgagacagctgaggccacgcgtctgaaacgtacagcaagaagacgttacacacgtcgtaaaaatcgtatttgctacttacaggaaattttttctaacgaaatggccaaggtagatgatagtttcttccatcgtctcgaagaatcttttctggttgaggaagataaaaaacacgaacgtcaccctatctttggcaatatcgtggatgaagtggcctatcatgaaaaataccctacgatttatcatcttcgcaagaagttggttgatagtacggacaaagcggatctgcgtttaatctatcttgcgttagcgcacatgatcaaatttcgtggtcatttcttaattgaaggtgatctgaatcctgataactctgatgtggacaaattgtttatacaattagtgcaaacctataatcagctgttcgaggaaaaccccattaatgcctctggagttgatgccaaagcgattttaagcgcgagactttctaagtcccggcgtctggagaatctgatcgcccagttaccaggggaaaagaaaaatggtctgtttggtaatctgattgccctcagtctggggcttaccccgaacttcaaatccaattttgacctggctgaggacgcaaagctgcagctgagcaaagatacttatgatgatgacctcgacaatctgctcgcccagattggtgaccaatatgcggatctgtttctggcagcgaagaatctttcggatgctatcttgctgtcggatattctgcgtgttaataccgaaatcaccaaagcgcctctgtctgcaagtatgatcaagagatacgacgagcaccaccaggacctgactcttcttaaggcactggtacgccaacagcttccggagaaatacaaagaaatattcttcgaccagtccaagaatggttacgcgggctacatcgatggtggtgcatcacaggaagagttctataaatttattaaaccaatccttgagaaaatggatggcacggaagagttacttgttaaacttaaccgcgaagacttgcttagaaagcaacgtacattcgacaacggctccatcccacaccagattcatttaggtgaacttcacgccatcttgcgcagacaagaagatttctatcccttcttaaaagacaatcgggagaaaatcgagaagatcctgacgttccgcattccctattatgtcggtcccctggcacgtggtaattctcggtttgcctggatgacgcgcaaaagtgaggaaaccatcaccccttggaactttgaagaagtcgtggataaaggtgctagcgcgcagtcttttatagaaagaatgacgaacttcgataaaaacttgcccaacgaaaaagtcctgcccaagcactctcttttatatgagtactttactgtgtacaacgaactgactaaagtgaaatacgttacggaaggtatgcgcaaacctgcctttcttagtggcgagcagaaaaaagcaattgtcgatcttctctttaaaacgaatcgcaaggtaactgtaaaacagctgaaggaagattatttcaaaaagatcgaatgctttgattctgtcgagatctcgggtgtcgaagatcgtttcaacgcttccttagggacctatcatgatttgctgaagataataaaagacaaagactttctcgacaatgaagaaaatgaagatattctggaggatattgttttgaccttgaccttattcgaagatagagagatgatcgaggagcgcttaaaaacctatgcccacctgtttgatgacaaagtcatgaagcaattaaagcgccgcagatatacggggtggggccgcttgagccgcaagttgattaacggtattagagacaagcagagcggaaaaactatcctggatttcctcaaatctgacggatttgcgaaccgcaattttatgcagcttatacatgatgattcgcttacattcaaagaggatattcagaaggctcaggtgtctgggcaaggtgattcactccacgaacatatagcaaatttggccggctctcctgcgattaagaaggggatcctgcaaacagttaaagttgtggatgaacttgtaaaagtaatgggccgccacaagccggagaatatcgtgatagaaatggcgcgcgagaatcaaacgacacaaaaaggtcaaaagaactcaagagagagaatgaagcgcattgaggaggggataaaggaacttggatctcaaattctgaaagaacatccagttgaaaacactcagctgcaaaatgaaaaattgtacctgtactacctgcagaatggaagagacatgtacgtggatcaggaattggatatcaatagactctcggactatgacgtagatcacattgtccctcagagcttcctcaaggatgattctatagataataaagtacttacgagatcggacaaaaatcgcggtaaatcggataacgtcccatcggaggaagtcgttaaaaagatgaaaaactattggcgtcaactgctgaacgccaagctgatcacacagcgtaagtttgataatctgactaaagccgaacgcggtggtcttagtgaactcgataaagcaggatttataaaacggcagttagtagaaacgcgccaaattacgaaacacgtggctcagatcctcgattctagaatgaatacaaagtacgatgaaaacgataaactgatccgtgaagtaaaagtcattaccttaaaatctaaacttgtgtccgatttccgcaaagattttcagttttacaaggtccgggaaatcaataactatcaccatgcacatgatgcatatttaaatgcggttgtaggcacggcccttattaagaaataccctaaactcgaaagtgagtttgtttatggggattataaagtgtatgacgttcgcaaaatgatcgcgaaatcagaacaggaaatcggtaaggctaccgctaaatactttttttattccaacattatgaatttttttaagaccgaaataactctcgcgaatggtgaaatccgtaaacggcctcttatagaaaccaatggtgaaacgggagaaatcgtttgggataaaggtcgtgactttgccaccgttcgtaaagtcctctcaatgccgcaagttaacattgtcaagaagacggaagttcaaacagggggattctccaaagaatctatcctgccgaagcgtaacagtgataaacttattgccagaaaaaaagattgggatccaaaaaaatacggaggctttgattcccctaccgtcgcgtatagtgtgctggtggttgctaaagtcgagaaagggaaaagcaagaaattgaaatcagttaaagaactgctgggtattacaattatggaaagatcgtcctttgagaaaaatccgatcgactttttagaggccaaggggtataaggaagtgaaaaaagatctcatcatcaaattaccgaagtatagtctttttgagctggaaaacggcagaaaaagaatgctggcctccgcgggcgagttacagaagggaaatgagctggcgctgccttccaaatatgttaattttctgtaccttgccagtcattatgagaaactgaagggcagccccgaagataacgaacagaaacaattattcgtggaacagcataagcactatttagatgaaattatagagcaaattagtgaattttctaagcgcgttatcctcgcggatgctaatttagacaaagtactgtcagcttataataaacatcgggataagccgattagagaacaggccgaaaatatcattcatttgtttaccttaaccaaccttggagcaccagctgccttcaaatatttcgataccacaattgatcgtaaacggtatacaagtacaaaagaagtcttggacgcaaccctcattcatcaatctattactggattatatgagacacgcattgatctttcacagctgggcggagacaagaagaaaaaactgaaactgcaccatcatcaccatcatcatcaccatcattgataactcgagaaagcttacataaaaaaccggccttggccccgccggttttttattatttttcttcctccgcatgttcaatccgctccataatcgacggatggctccctctgaaaattttaacgagaaacggcgggttgacccggctcagtcccgtaacggccaagtcctgaaacgtctcaatcgccgcttcccggtttccggtcagctcaatgccgtaacggtcggcggcgttttcctgataccgggagacggcattcgtaatc

SEQ ID NO: 43 - DNA, 17 bp, Artificial Sequence
  pRF694 forward
gaattcgcggccgcacg

SEQ ID NO: 44 - DNA, 29 bp, Artificial Sequence
  pRF694 reverse
gattacgaatgccgtctcccggtatcagg

SEQ ID NO: 45 - DNA, 1365 bp, Artificial Sequence
  rghR2 ET gRNA cassette
ggcggcgttttcctgataccgggagacggcattcgtaatcgtatgaggaactgatggcatctgcaggctatatcagcgcgtctacagtccaggaagcaagaagcagctatgattccatttacgacatcgtgtcacagtacgatttagaggacctttctctgtttgacagcgaaaagtggaaggtgctttcaaaaaaagacatcgaaaacctggacaaatatttcgactttctcgtgcaggaagcaagcagccgaaacaaaaactgaatacttctccgcggcacactctcctctctatcattttcgtctgtttacgatcctgctgttattttatcccttatgttaacttttgtcaatatttttcctgtctaagtatttcctatagtcaacatttgtattaaaatgttcatatcatgaatttgcgggggggatggcgatgacaaggttcggcgagcggctcaaagagctgagggaacaaagaagcctgtcggttaatcagcttgccatgtatgccggtgtgagcgccgcagccatttccagaatcgaaaacggccaccgcggcgttcccaagcccgcgacgatcagaaaattggccgaggctctgaaaatgccgtacgagcagctcatggatattgccggttatatgagagctgacgagattcgcgaacagccgcgcggctatgtcacgatgcaggagatcgcggccaagcacggcgtcgaagacctgtggctgtttaaacccgagaaatgggactgtttgtcccgcgaagacctgctcaacctcgaacagtattttcattttttggttaatgaagcgaagaagcgccaatcataaaaagccgaatttcccttttaggagaagttcggcttttttcggctgccttaagcggcatccggattcggcgtcttgcctttatgatgcttaacggggctcagcgcacgctcgagccatcccatgaacagatcggcgatgatcgccatcagcgccgtcgggatcgcgcctgctagaatgatcgctgttccgttggtcgcgtttgatcctcgctgataaacagctgacatcaactaaaagcttcattaaatactttgaaaaaagttgttgacttaaaagaagctaaatgttatagtaataaaaaatggctgcggctctggaaagttttagagctagaaatagcaagttaaaataaggctagtccgttatcaacttgaaaaagtggcaccgagtcggtgcgactcctgttgatagatccagtaatgacctcagaactccatctggatttgttcagaacgctcggttgccgccgggcgttttttattggtgagaatgaattcgcggccgcacgcgtccatggggatccccgcgggt

SEQ ID NO: 46 - DNA, 1000 bp, Artificial Sequence
  rghR2 editing template
gtatgaggaactgatggcatctgcaggctatatcagcgcgtctacagtccaggaagcaagaagcagctatgattccatttacgacatcgtgtcacagtacgatttagaggacctttctctgtttgacagcgaaaagtggaaggtgctttcaaaaaaagacatcgaaaacctggacaaatatttcgactttctcgtgcaggaagcaagcagccgaaacaaaaactgaatacttctccgcggcacactctcctctctatcattttcgtctgtttacgatcctgctgttattttatcccttatgttaacttttgtcaatatttttcctgtctaagtatttcctatagtcaacatttgtattaaaatgttcatatcatgaatttgcgggggggatggcgatgacaaggttcggcgagcggctcaaagagctgagggaacaaagaagcctgtcggttaatcagcttgccatgtatgccggtgtgagcgccgcagccatttccagaatcgaaaacggccaccgcggcgttcccaagcccgcgacgatcagaaaattggccgaggctctgaaaatgccgtacgagcagctcatggatattgccggttatatgagagctgacgagattcgcgaacagccgcgcggctatgtcacgatgcaggagatcgcggccaagcacggcgtcgaagacctgtggctgtttaaacccgagaaatgggactgtttgtcccgcgaagacctgctcaacctcgaacagtattttcattttttggttaatgaagcgaagaagcgccaatcataaaaagccgaatttcccttttaggagaagttcggcttttttcggctgccttaagcggcatccggattcggcgtcttgcctttatgatgcttaacggggctcagcgcacgctcgagccatcccatgaacagatcggcgatgatcgccatcagcgccgtcgggatcgcgcctgctagaatgatcgctgttccgttggtcgcgtttgatcc

SEQ ID NO: 47 - DNA, 285 bp, Artificial Sequence
  rghR2 gRNA expression cassette
tcgctgataaacagctgacatcaactaaaagcttcattaaatactttgaaaaaagttgttgacttaaaagaagctaaatgttatagtaataaaaaatggctgcggctctggaaagttttagagctagaaatagcaagttaaaataaggctagtccgttatcaacttgaaaaagtggcaccgagtcggtgcgactcctgttgatagatccagtaatgacctcagaactccatctggatttgttcagaacgctcggttgccgccgggcgttttttattggtgagaat

SEQ ID NO: 48 - DNA, 25 bp, Artificial Sequence
  rghR2 cassette forward primer
ggcggcgttttcctgataccgggag

SEQ ID NO: 49 - DNA, 20 bp, Artificial Sequence
  rghR2 cassette reverse primer
acccgcggggatccccatgg

SEQ ID NO: 50 - DNA, 6393 bp, Artificial Sequence
  plasmid pBL.comK
aagcttcatatgcaagggtttattgttttctaaaatctgattaccaattagaatgaatatttcccaaatattaaataataaaacaaaaaaattgaaaaaagtgtttccaccattttttcaatttttttataatttttttaatctgttatttaaatagtttatagttaaatttacattttcattagtccattcaatattctctccaagataactacgaactgctaacaaaattctctccctatgttctaatggagaagattcagccactgcatttcccgcaatatcttttggtatgattttacccgtgtccatagttaaaatcatacggcataaagttaatatagagttggtttcatcatcctgataattatctattaattcctctgacgaatccataatggctcttctcacatcagaaaatggaatatcaggtagtaattcctctaagtcataatttccgtatattcttttattttttcgttttgcttggtaaagcattatggttaaatctgaatttaattccttctgaggaatgtatccttgttcataaagctcttgtaaccattctccataaataaattcttgtttgggaggatgattccacggtaccatttcttgctgaataataattgttaattcaatatatcgtaagttgcttttatctcctattttttttgaaataggtctaattttttgtataagtatttctttactttgatctgtcaatggttcagatacgacgactaaaaagtcaagatcactatttggttttagtccactctcaactcctgatccaaacatgtaagtaccaataaggttattttttaaatgtttccgaagtatttttttcactttattaatttgttcgtatgtattcaaatatatcctcctcactattttgattagtacctattttatatccatagttgttaattaaataaacttaatttagtttatttatggatttcattggcttctaaattttttatctagataataattattttagttaattttattctagattatatatgatatgatctttcatttccataaaactaaagtaagtgtaaacctattcattgttttaaaaatatctcttgccagtcacgttacgttattagttatagttattataacatgtattcacgaacgggcgcgccggtatccgcgcttcttgagcactatttattcaaagccgctccagatcaatagcgctttttcagctccctgaggatgaattcgtatatcagctgattccggtcttctttcggatagagcataaattcctgtttcttctgcatggggtttccttcaatcctgtcgataaattttgttctcagccatgccgttcggtaaacctggttttcgaaagatgagatggatacgggcagctccagcgtttccccgttgacaaacgtgacaaacgtgttgtcatactttgccgcgcaaaactcgtgaacatgcgcatgggaaagccacccgcactgaggacgagttgaggaaaatgtggggaaaagaaaaatgttgtttgagtgatccaccatgatcggcggtttatgggaaactttaatgacttcatatgtgcccgcttttcttcccgcatagctcgatccgaaatagcggcagcttctttcgataatttgaaacggcttcatattgacgcggaaagtcctgtcggtctcaagtatttttgaggcggatttctccccctcacccagaggcaggacagccattgtcgaactgtttacttcatacgtatcctttgtcatatcctctgtgctcatgtgatttcccccttaaaaataaattcattcaaatacagatgcattttatttcatatagtaagtacatcacctattagtttgttgtttaaacaaactaacttattttcatcttatataacctcgtcagtattttcaatattttttttagttttttatgaacacattagatttaataaagggaagattcgctatgtactatgttgatacttaatttaaagattaaacaaatggagtggatgaagtggatatcgctgatcaaacctttgtcaaaaaagtaaatcaaaagttattattaaaagaaatccttaaaaattcacctatttcaagagcaaaattatctgaaatgactggattaaataaatcaactgtctcatcacaggtaaacacgttaatgaaagaaagtatggtatttgaaataggtcaaggacaatcaagtggcggaagaagacctgtcatgcttgtttttaataaaaaggcaggatactccgttggaatagatgttggtgtggattatattaatggcattttaacagaccttgaaggaacaatcgttcttgatcaataccgccatttggaatccaattctccagaaataacgaaagacattttgattgatatgattcatcactttattacgcaaatgccccaatctccgtacgggtttattggtataggtacttgcgtgcctggactcattgataaagatcaaaaaattgttttcactccgaactccaactggagagatattgacttaaaatcttcgatacaagagaagtacaatgtgtctgtttttattgaaaatgaggcaaatgctggcgcatatggagaaaaactatttggagctgcaaaaaatcacgataacattatttacgtaagtatcagcacaggaatagggatcggtgttattatcaacaatcatttatatagaggagtaagcggcttctctggagaaatgggacatatgacaatagactttaatggtcctaaatgcagttgcggaaaccgaggatgctgggaattgtatgcttcagagaaggctttatttaaatctcttcagaccaaagagaaaaaactgtcctatcaagatatcataaacctcgcccatctgaatgatatcggaaccttaaatgcattacaaaattttggattctatttaggaataggccttaccaatattctaaatactctcaacccacaagccgtaattttaagaaatagcataattgaatcgcatcctatggttttaaattcaatgagaagtgaagtatcatcaagggtttattcccaattaggcaatagctatgaattattgccatcttccttaggacagaatgcaccggcattaggaatgtcctccattgtgattgatcattttctggacatgattacaatgtaattttttatggaatggacagctcatctttaaagatgagtttttttattctaggagtatttctgaagcaatagtgacatggcaccttctcatatgaaaaaggagttctaaaataaaaatctcctttttcatgtgcaaattatttttctttataacgaaaatatctaaatgacaatgcatatgcaagaggggatcacataaatatatattttaaaaatatcccactttatccaattttcgtttgttgaactaatgggtgctttagttgaagaataaaagaccacattaaaaaatgtggtcttttgtgtttttttaaaggatttgagcgtagcgaaaaatccttttctttcttatcttgatactatatagaaacaacatcatttttcaaaattaggtcaaagccttgtgtatcaagggtttgatggttctttgacaggtaaaaactccttctgctattattaaatactatatagaaacaacatcatttttcaaaattaggtcaaagccttgtgtatcaagggtttgatggttctttgacaggtaaaaactccttctgctattattaaggtgtcgaatcaaaataatagaatgctagagaactagctcagaaggagtttttttgttgatttattcatctgaaaatgattatagcatcctcgaagataaaaccgcaacaggtaaaaagcgggattggaaggggaaaaagagacggacgaacctcatggcggagcattacgaagcgttagagagtaagattggggcaccttactatggcaaaaaggctgaaaaactaattagttgtgcagagtatctttcgtttaagagagacccggagacgggcaagttaaaactgtatcaagcccatttttgtaaagtgaggttatgtccgatgtgtgcgtggcgcaggtcgttaaaaattgcttatcacaataagttgatcgtagaggaagccaatagacagtacggctgcggatggatttttctcacgctgacgattcgaaatgtaaagggagaacggctgaagccacaaatttctgcgatgatggaaggctttaggaaactgttccagtacaaaaaagtaaaaacttcggttcttggatttttcagagctttagagattaccaaaaatcatgaagaagatacatatcatcctcattttcatgtgttgataccagtaaggaaaaattattttgggaaaaactatattaagcaggcggagtggacgagcctttggaaaaaggcgatgaaattggattacactccaattgtcgatattcgtcgagtgaaaggtaaagctaagattgacgctgaacagattgaaaacgatgtgcggaacgcaatgatggagcaaaaagctgttctcgaaatctctaaatatccggttaaggatacggatgttgtgcgcggtaataaggtgactgaagacaatctgaacacggtgctttacttggatgatgcgttggcagctcgaaggttaattggatacggtggcattttgaaggagatacataaagagctgaatcttggtgatgcggaggacggcgatctggtcaagattgaggaagaagatgacgaggttgcaaatggtgcatttgaggttatggcttattggcatcctggcattaaaaattacataatcaaataaaaaaagcagacctttagaaggcctgcttttttaactaacccatttgtattgtgttgaaatatgttttgtatggtgcactctcagtacaatctgctctgatgccgcatagttaagccagccccgacacccgccaacacccgctgacgcgccctgacgggcttgtctgctcccggcatccgcttacagacaagctgtgaccgtctccgggagctgcatgtgtcagaggttttcaccgtcatcaccgaaacgcgcgagacgaaagggcctcgtgatacgcctatttttataggttaatgtcatgataataatggtttcttagcgattcacaaaaaataggcacacgaaaaacaagttaagggatgcagtttatgcatcccttaacttaaaatactaaaaatgcccatattttttcctccttataaaattagtataattatagcacgagatctaaaaggatctaggtgaagatcctttttgataatctcatgaccaaaatcccttaacgtgagttttcgttccactgagcgtcagaccccgtagaaaagatcaaaggatcttcttgagatcctttttttctgcgcgtaatctgctgcttgcaaacaaaaaaaccaccgctaccagcggtggtttgtttgccggatcaagagctaccaactctttttccgaaggtaactggcttcagcagagcgcagataccaaatactgttcttctagtgtagccgtagttaggccaccacttcaagaactctgtagcaccgcctacatacctcgctctgctaatcctgttaccagtggctgctgccagtggcgataagtcgtgtcttaccgggttggactcaagacgatagttaccggataaggcgcagcggtcgggctgaacggggggttcgtgcacacagcccagcttggagcgaacgacctacaccgaactgagatacctacagcgtgagctatgagaaagcgccacgcttcccgaagggagaaaggcggacaggtatccggtaagcggcagggtcggaacaggagagcgcacgagggagcttccagggggaaacgcctggtatctttatagtcctgtcgggtttcgccacctctgacttgagcgtcgatttttgtgatgctcgtcaggggggcggagcctatggaaaaacgccagcaacgcggcctttttacggttcctggccttttgctggccttttgctcacatgttctttcctgcgttatcccctgattctgtggataaccgtattaccgcctttgagtgagctgataccgctcgccgcagccgaacgaccgagcgcagcgagtcagtgagcgaggaagcggaagagcgcccaatacgcaaaccgcctctccccgcgcgttggccgattcattaatgcagctggcacgacaggtttcccgactggaaagcgggcagtgagcgcaacgcaattaatgtgagttagctcactcattaggcaccccaggctttacactttatgcttccggctcgtatgttgtgtggaattgtgagcggataacaatttcacacaggaaacagctatgaccatgattacgccggatcc

SEQ ID NO: 51 - DNA, 1069 bp, Bacillus licheniformis
cggcatcaagtggatattcccggaagcctcgctattttaagctgtgacaaccagccgatcagcgaagtgctcggcatttcaacaattgaaatcaatataaaggaaatggggaagcgcgcgtttcgccttctgcaaaaaagaatcggcggcgccgggccggaaaaactgactgttccttacaagctgatcaaaagggcgactgtgtaatcaaaacatcaatctttttccagacagtgatcaaaattcgacatttttcatcaaaaacgtcaaaataaattgacgcgctttcatgagttttgtacgatatgagagattgatgacaaaaaggagctgaggatcgtgaacagatcctttaccgttgaaaaggtactcaacaacaacgttttaatcgctctccatgatgattacagagaagttgtcttgattggcaaaggaatcggttttggtaaaaagcgcggagatcttatcgaacatgagaactacgaaaaaatgtttatcctggaaaatgataaggaacaatcgcagtataagaagctcctcacttatgtcgatgaaaaaatggttgatatcgccaatgatgtcatctaccatatcgcgcaaaaaatcggccagccgctgaacgaacacattcatgtcgccctgacggaccatatcgcatttgcagttaagcgtctagaaaagggatttgatatgaaaaatccgtttttgcttgagacggaatcgctttatccgaaggaatacgaagtcgccaaggaagccgtcgatatgattaatgaaaaatccgacattcagctgcctgaaggtgaaatcgggttcatcgcgcttcatatccacagtgcgatgacaaaccgcccgctttctgaagtcaatcagcattcacaactgatctccaggcttgtccaggtcatcgaagattcattccagatgcaagtcaacagggaaagcgtgaactatttgcggctgatcaggcacttgcgctttacgattgacaggataaaacgggacgagccgattcaggaaccggaaaaattaatgttgttgttgaaaacggaatatccgctgtgttaca

SEQ ID NO: 52 - DNA, 20 bp, Artificial Sequence
  glcT locus forward primer
cggcatcaagtggatattcc

SEQ ID NO: 53 - DNA, 20 bp, Artificial Sequence
  glcT locus reverse primer
tgtaacacagcggatattcc

SEQ ID NO: 54 - DNA, 20 bp, Artificial Sequence
  glcT locus forward sequencing primer
tgaggatcgtgaacagatcc

SEQ ID NO: 55 - protein, 281 aa, Artificial Sequence
  glcT L67F
VNRSFTVEKVLNNNVLIALHDDYREVVLIGKGIGFGKKRGDLIEHENYEKMFILENDKEQSQYKKLFTYVDEKMVDIANDVIYHIAQKIGQPLNEHIHVALTDHIAFAVKRLEKGFDMKNPFLLETESLYPKEYEVAKEAVDMINEKSDIQLPEGEIGFIALHIHSAMTNRPLSEVNQHSQLISRLVQVIEDSFQMQVNRESVNYLRLIRHLRFTIDRIKRDEPIQEPEKLMLLLKTEYPLCYNTAWKMIKILQQALKKPVHEAEAVYLTLHLYRLTNKIS

SEQ ID NO: 56 - DNA, 846 bp, Artificial Sequence
  glcT ORF encoding L67F
gtgaacagatcctttaccgttgaaaaggtactcaacaacaacgttttaatcgctctccatgatgattacagagaagttgtcttgattggcaaaggaatcggttttggtaaaaagcgcggagatcttatcgaacatgagaactacgaaaaaatgtttatcctggaaaatgataaggaacaatcgcagtataagaagctcttcacttatgtcgatgaaaaaatggttgatatcgccaatgatgtcatctaccatatcgcgcaaaaaatcggccagccgctgaacgaacacattcatgtcgccctgacggaccatatcgcatttgcagttaagcgtctagaaaagggatttgatatgaaaaatccgtttttgcttgagacggaatcgctttatccgaaggaatacgaagtcgccaaggaagccgtcgatatgattaatgaaaaatccgacattcagctgcctgaaggtgaaatcgggttcatcgcgcttcatatccacagtgcgatgacaaaccgcccgctttctgaagtcaatcagcattcacaactgatctccaggcttgtccaggtcatcgaagattcattccagatgcaagtcaacagggaaagcgtgaactatttgcggctgatcaggcacttgcgctttacgattgacaggataaaacgggacgagccgattcaggaaccggaaaaattaatgttgttgttgaaaacggaatatccgctgtgttacaatactgcttggaagatgatcaagatcttgcagcaagcgctcaagaaaccggttcatgaggcagaagccgtttatttgacattgcatttgtaccgtttgactaataaaatttcataa

SEQ ID NO: 57 - DNA, 1164 bp, Bacillus licheniformis
gcgaatcgaaaacggaaagcgcggcgtgccgaagccggcgacgatcagaaaactggcggacgctttgaaagtcccgtatgaggaactgatggcatctgcaggctatatcagcgcgtctacagtccaggaagcaagaagcagctatgattccatttacgacatcgtgtcacagtacgatttagaggacctttctctgtttgacagcgaaaagtggaaggtgctttcaaaaaaagacatcgaaaacctggacaaatatttcgactttctcgtgcaggaagcaagcagccgaaacaaaaactgaatacttctccgcggcacactctcctctctatcattttcgtctgtttacgatcctgctgttattttatcccttatgttaacttttgtcaatatttttcctgtctaagtatttcctatagtcaacatttgtattaaaatgttcatatcatgaatttgcgggggggatggcgatgacaaggttcggcgagcggctcaaagagctgagggaacaaagaagcctgtcggttaatcagcttgccatgtatgccggtgtgagcgccgcagccatttccagagccgcagccatttccagaatcgaaaacggccaccgcggcgttcccaagcccgcgacgatcagaaaattggccgaggctctgaaaatgccgtacgagcagctcatggatattgccggttatatgagagctgacgagattcgcgaacagccgcgcggctatgtcacgatgcaggagatcgcggccaagcacggcgtcgaagacctgtggctgtttaaacccgagaaatgggactgtttgtcccgcgaagacctgctcaacctcgaacagtattttcattttttggttaatgaagcgaagaagcgccaatcataaaaagccgaatttcccttttaggagaagttcggcttttttcggctgccttaagcggcatccggattcggcgtcttgcctttatgatgcttaacggggctcagcgcacgctcgagccatcccatgaacagatcggcgatgatcgccatcagcgccgtcgggatcgcgcctgctagaatgatcgctgttccgttggtcgcgtttgatcccctgacaatgatatccccgaggccgcctgcgccgacaaacgtgccgatggccgtaatgccgatcgcgatga

SEQ ID NO: 58 - DNA, 20 bp, Artificial Sequence
  rghR2 locus forward primer
gcgaatcgaaaacggaaagc

SEQ ID NO: 59 - DNA, 20 bp, Artificial Sequence
  rghR2 locus reverse primer
tcatcgcgatcggcattacg

SEQ ID NO: 60 - DNA, 20 bp, Artificial Sequence
  rghR2 locus sequencing primer
tttcgactttctcgtgcagg

SEQ ID NO: 61 - DNA, 1146 bp, Bacillus licheniformis
gcgaatcgaaaacggaaagcgcggcgtgccgaagccggcgacgatcagaaaactggcggacgctttgaaagtcccgtatgaggaactgatggcatctgcaggctatatcagcgcgtctacagtccaggaagcaagaagcagctatgattccatttacgacatcgtgtcacagtacgatttagaggacctttctctgtttgacagcgaaaagtggaaggtgctttcaaaaaaagacatcgaaaacctggacaaatatttcgactttctcgtgcaggaagcaagcagccgaaacaaaaactgaatacttctccgcggcacactctcctctctatcattttcgtctgtttacgatcctgctgttattttatcccttatgttaacttttgtcaatatttttcctgtctaagtatttcctatagtcaacatttgtattaaaatgttcatatcatgaatttgcgggggggatggcgatgacaaggttcggcgagcggctcaaagagctgagggaacaaagaagcctgtcggttaatcagcttgccatgtatgccggtgtgagcgccgcagccatttccagaatcgaaaacggccaccgcggcgttcccaagcccgcgacgatcagaaaattggccgaggctctgaaaatgccgtacgagcagctcatggatattgccggttatatgagagctgacgagattcgcgaacagccgcgcggctatgtcacgatgcaggagatcgcggccaagcacggcgtcgaagacctgtggctgtttaaacccgagaaatgggactgtttgtcccgcgaagacctgctcaacctcgaacagtattttcattttttggttaatgaagcgaagaagcgccaatcataaaaagccgaatttcccttttaggagaagttcggcttttttcggctgccttaagcggcatccggattcggcgtcttgcctttatgatgcttaacggggctcagcgcacgctcgagccatcccatgaacagatcggcgatgatcgccatcagcgccgtcgggatcgcgcctgctagaatgatcgctgttccgttggtcgcgtttgatcccctgacaatgatatccccgaggccgcctgcgccgacaaacgtgccgatggccgtaatgccgatcgcgatga

SEQ ID NO: 62 - DNA, 58 bp, Bacillus subtilis
acagaatagtcttttaagtaagtctactctgaatttttttaaaaggagagggtaaaga

SEQ ID NO: 63 - DNA, 57 bp, Artificial Sequence
  aprE mod-5' UTR
acagaatagtcttttaagtaagtctactctgaatttttttaaaaggagagggtaaag

SEQ ID NO: 64 - DNA, 6208 bp, Artificial Sequence
  WT 5' UTR expression construct
ggctatgacgaaacgattgcagcctatgaggcgagtctcgaaaagctcggacttgactaccttgatttatacctgatccactggcctgttgaaggacgctacaaagcggcgtggaaagcgcttgaaacactttatgaacaaggacgcgtaaaagcaatcggagtgagcaattttcagattcaccatctggaagacttgctgaaagatgccgccgtcaaaccggcgatcaaccaggttgagtatcatccgcggctgacgcagaaagagctgcaagcgttttgccgtgcgcacggcatccagctgcaagcatggtcgccgctgatgcaaggccaattgctcagccatccactgctgaaagatatcgcggacaagtacggcaagacaccggcccaagtcattttgcgctgggatttgcaaaacggggtcgttacgattccgaagtcgactaaagcggagcggattgcccaaaacgcggacatatttgattttgaactgaccaccgaggaaatgaagcaaattgacgcgctgaatgaaaacacccgtgtcggccctgatcccgataactttgacttttaacaaaacggccccgttcgacattcgaacggggctttaattgaattgtgcggttacaccgccggactccatcatcatcagttcttttttcatatccaatccgccccggtatcccgtgagctgcccgcttttaccgataacccgatggcaaggcaccaccattaacagcggatttgcgccgatcgccgcgcctactgcccgcacagcggcctgcttttcaatatgctcggcgatatcggaataggagcaagtgctgccgtaagggatttcggagagcgccttccacactgccagctgaaaaggcgtgccggcaaggtcgacaggaaagctgaaatgagttcgcttgccgttcaaatacgcctgcagctgctcggcgtattctgccaatcctttgtcatcccgaatgaaaactggctgtgtaaatcttttttcagcccaagcggccaaatcctcgaagccttgattccatccccctgtaaaacagagcccgcgggcagtcgccccaatgtgaatctgccaacctcggcaaataagcgtacgccagtatacgatttgatcgtccatatgtttacctccgtttcatttgccggtacgacgtcggcgattgcccagtcttctttttaaacaaagaggcaaaatattccgcattcgcaatgcctaccattgaagcgatttctgcgatcgatcgttctgaatgagcaagcaaatcgaccgctttctcaatccttttctgcaggatgtattctgccggcgagacgcctttgattcgtttaaatgtccgctgcaggtgaaaagggctgatatggcacctgtcagccaaagcttgcagagacagcggatcgcgataagattcctcgatgatttccaccacacgctgtgccagctcttcatccggcagcagcgccccggccggattgcagcgtttgcaggggcggtacccttctgataaagcatcttttgcattgaaaaagatctgcacattgtcgatttgcggaactctcgatttgcaggaagggcggcaaaatatgccggtcgttttgaccgcgtaataaaaaactccgtcataggcggaatcgttttccgtaatcgcccgccacatttcaggcgtcaatcgtgatttgctgttcatatcttcaccccgatctatgtcagtataacctatatgacagccggaggtggagaggcggagaacggcacagcaagaagacaaagaagaagagagactgttgcctggacctccgaaacgcgctacaattcatttacaacacaggatggggtgagaatattgccggaatcagtgaagcaggcctcctaaaataaaaatctatattttaggaggtaaaacatgaattttcaaacaatcgagcttgacacatggtatagaaaatcttattttgaccattacatgaaggaagcgaaatgttctttcagcatcacggcaaacgtcaatgtgacaaatttgctcgccgtgctcaagaaaaagaagctcaagctgtatccggcttttatttatatcgtatcaagggtcattcattcgcgccctgagtttagaacaacgtttgatgacaaaggacagctgggttattgggaacaaatgcatccgtgctatgcgatttttcatcaggacgaccaaacgttttccgccctctggacggaatactcagacgatttttcgcagttttatcatcaatatcttctggacgccgagcgctttggagacaaaaggggcctttgggctaagccggacatcccgcccaatacgttttcagtttcttctattccatgggtgcgcttttcaaacttcaatttaaaccttgataacagcgaacacttgctgccgattattacaaacgggaaatacttttcagaaggcagggaaacatttttgcccgtttccttgcaagttcaccatgcagtgtgtgacggctatcatgccggcgcttttataaacgagttggaacggcttgccgccgattgtgaggagtggcttgtgtgacagaggaaaggccgatatgattcggccttttttatatgtacttcttagcgggtctcttaacccccctcgaggtcgctgataaacagctgacatcaatatcctattttttcaaaaaatattttaaaaagttgttgacttaaaagaagctaaatgttatagtaataaaacagaatagtcttttaagtaagtctactctgaatttttttaaaaggagagggtaaagaatgaaacaacaaaaacggctttacgcccgattgctgacgctgttatttgcgctcatcttcttgctgcctcattctgcagctagcgcagccgcaccgtttaacggtaccatgatgcagtattttgaatggtacttgccggatgatggcacgttatggaccaaagtggccaatgaagccaacaacttatccagccttggcatcaccgctctttggctgccgcccgcttacaaaggaacaagccgcagcgacgtagggtacggagtatacgacttgtatgacctcggcgaattcaatcaaaaagggaccgtccgcacaaaatatggaacaaaagctcaatatcttcaagccattcaagccgcccacgccgctggaatgcaagtgtacgccgatgtcgtgttcgaccataaaggcggcgctgacggcacggaatgggtggacgccgtcgaagtcaatccgtccgaccgcaaccaagaaatctcgggcacctatcaaatccaagcatggacgaaatttgattttcccgggcggggcaacacctactccagctttaagtggcgctggtaccattttgacggcgttgattgggacgaaagccgaaaattaagccgcatttacaaattcaggggcatcggcaaagcgtgggattggccggtagacacagaaaacggaaactatgactacttaatgtatgccgaccttgatatggatcatcccgaagtcgtgaccgagctgaaaaactgggggaaatggtatgtcaacacaacgaacattgatgggttccggcttgatgccgtcaagcatattaagttcagtttttttcctgattggttgtcgtatgtgcgttctcagactggcaagccgctatttaccgtcggggaatattggagctatgacatcaacaagttgcacaattacattacgaaaacaaacggaacgatgtctttgtttgatgccccgttacacaacaaattttataccgcttccaaatcagggggcgcatttgatatgcgcacgttaatgaccaatactctcatgaaagatcaaccgacattggccgtcaccttcgttgataatcatgacaccgaacccggccaagcgcttcagtcatgggtcgacccatggttcaaaccgttggcttacgcctttattctaactcggcaggaaggatacccgtgcgtcttttatggtgactattatggcattccacaatataacattccttcgctgaaaagcaaaatcgatccgctcctcatcgcgcgcagggattatgcttacggaacgcaacatgattatcttgatcactccgacatcatcgggtggacaagggaaggggtcactgaaaaaccaggatccgggctggccgcactgatcaccgatgggccgggaggaagcaaatggatgtacgttggcaaacaacacgctggaaaagtgttctatgaccttaccggcaaccggagtgacaccgtcaccatcaacagtgatggatggggggaattcaaagtcaatggcggttcggtttcggtttgggttcctagaaaaacgacctaaaagcttctcgaggttaacagaggacggatttcctgaaggaaatccgtttttttatttttaacatctctcactgctgtgtgattttactcacggcatttggaacgccggctctcaacaaactttctgtagtgaaaatcatgaaccaaacggatcgtcggcctgattaacagctgaaagctgccgatcacaaacatccatagtcccgccggcttcagttcctcggagaaaaagcagaagctcccgacaaggaataaaaggccgatgagaaaatcgtttaatgtatgtagaactttgtatctttttttgaaaaagagttcatatcgattgttattgttttgcggcattgcttgatcactccaatccttttatttaccctgccggaagccggagtgaaacgccggtatacataggatttatgaattaggaaaacatatggggaaataaaccatccaggagtgaaaaatatgcggttattcatatgtgcatcgtgcctgttcggcttgattgttccgtcatttgaaacgaaagcgctgacgtttgaagaattgccggttaaacaagcttcaaaacaatgggaagttcaaatcggtaaagccgaagccggaaacggaatggcgaaaccggaaaaaggagcgtttcatacttatgctgtcgaaatcaaaaacattggacacgatgtggcttcggcggaaatttttgtctatcggaacgagcctaattcttcaacgaaattttcgctttggaacattcctcacgaaaatccggtttctttagccaaaagcttaaatcacggaagctctgtcaagcaccgcaatctgcttatggcagagaatgcgaccgaattggaagtggacatgatttggacggaaaaaggaagcgaaggcagacttttaaaggaaacgttcattttcaagggagatgaatcatgaagaaaaaatggccgttcatcgtcaacggtctttttttaatgacttaggcagccgatcgttcggccatacgatatcgaagcgacctcgaaccagcagagctcgtcacaaaacatttgcatttaaagaaaaatacaggatgttttcaccaatatttttctcaatgatgatacactattgacaagctgctactttgggagggtgtttccatagatgccgatgaagcaaaaacaccaaatgtgtcatgagagctctctctaatcgatataaaagtagggtgaaccggggttgtcaatctgtaaaagatctttttttatcccgtgatacgcttttggaattctgaatcttcaagaaagtccccagccttttgctgatcaatcgagaacaaaggatgatacatatgaaaagaatagataaaatctaccatcagctgctggataattttcgcgaaaagaatatcaatcagcttttaaagatacaagggaattcggctaaagaaatcgccgggcagctgcaaatggagcgttccaatgtcagctttgaattaaacaatctggttcgggccaaaaaggtgatcaagattaaaacgttccccgtccgctacatcccggtggaaattgttgaaaacgtcttgaacatcaaatggaattcagagttgatggaggttgaagaactgaggcggctggctgacggccaaaaaaagccggcgcgcaatatatccgccgatcccctcgagctcatgatcggggctaaagggagcttgaaaaaggcaatttctcaggcgaaagcggcagtcttttatcctccgcacggcttgcatatgctgctgctcgggccgacgggttcggggaaatcgctgtttgcgaatcggatctaccagttcgccgtttattctgacatattgaagcccgattccccgttcatcacattcaactgtgcag

SEQ ID NO: 65 - DNA, 6207 bp, Artificial Sequence
  Mod 5' UTR expression construct
ggctatgacgaaacgattgcagcctatgaggcgagtctcgaaaagctcggacttgactaccttgatttatacctgatccactggcctgttgaaggacgctacaaagcggcgtggaaagcgcttgaaacactttatgaacaaggacgcgtaaaagcaatcggagtgagcaattttcagattcaccatctggaagacttgctgaaagatgccgccgtcaaaccggcgatcaaccaggttgagtatcatccgcggctgacgcagaaagagctgcaagcgttttgccgtgcgcacggcatccagctgcaagcatggtcgccgctgatgcaaggccaattgctcagccatccactgctgaaagatatcgcggacaagtacggcaagacaccggcccaagtcattttgcgctgggatttgcaaaacggggtcgttacgattccgaagtcgactaaagcggagcggattgcccaaaacgcggacatatttgattttgaactgaccaccgaggaaatgaagcaaattgacgcgctgaatgaaaacacccgtgtcggccctgatcccgataactttgacttttaacaaaacggccccgttcgacattcgaacggggctttaattgaattgtgcggttacaccgccggactccatcatcatcagttcttttttcatatccaatccgccccggtatcccgtgagctgcccgcttttaccgataacccgatggcaaggcaccaccattaacagcggatttgcgccgatcgccgcgcctactgcccgcacagcggcctgcttttcaatatgctcggcgatatcggaataggagcaagtgctgccgtaagggatttcggagagcgccttccacactgccagctgaaaaggcgtgccggcaaggtcgacaggaaagctgaaatgagttcgcttgccgttcaaatacgcctgcagctgctcggcgtattctgccaatcctttgtcatcccgaatgaaaactggctgtgtaaatcttttttcagcccaagcggccaaatcctcgaagccttgattccatccccctgtaaaacagagcccgcgggcagtcgccccaatgtgaatctgccaacctcggcaaataagcgtacgccagtatacgatttgatcgtccatatgtttacctccgtttcatttgccggtacgacgtcggcgattgcccagtcttctttttaaacaaagaggcaaaatattccgcattcgcaatgcctaccattgaagcgatttctgcgatcgatcgttctgaatgagcaagcaaatcgaccgctttctcaatccttttctgcaggatgtattctgccggcgagacgcctttgattcgtttaaatgtccgctgcaggtgaaaagggctgatatggcacctgtcagccaaagcttgcagagacagcggatcgcgataagattcctcgatgatttccaccacacgctgtgccagctcttcatccggcagcagcgccccggccggattgcagcgtttgcaggggcggtacccttctgataaagcatcttttgcattgaaaaagatctgcacattgtcgatttgcggaactctcgatttgcaggaagggcggcaaaatatgccggtcgttttgaccgcgtaataaaaaactccgtcataggcggaatcgttttccgtaatcgcccgccacatttcaggcgtcaatcgtgatttgctgttcatatcttcaccccgatctatgtcagtataacctatatgacagccggaggtggagaggcggagaacggcacagcaagaagacaaagaagaagagagactgttgcctggacctccgaaacgcgctacaattcatttacaacacaggatggggtgagaatattgccggaatcagtgaagcaggcctcctaaaataaaaatctatattttaggaggtaaaacatgaattttcaaacaatcgagcttgacacatggtatagaaaatcttattttgaccattacatgaaggaagcgaaatgttctttcagcatcacggcaaacgtcaatgtgacaaatttgctcgccgtgctcaagaaaaagaagctcaagctgtatccggcttttatttatatcgtatcaagggtcattcattcgcgccctgagtttagaacaacgtttgatgacaaaggacagctgggttattgggaacaaatgcatccgtgctatgcgatttttcatcaggacgaccaaacgttttccgccctctggacggaatactcagacgatttttcgcagttttatcatcaatatcttctggacgccgagcgctttggagacaaaaggggcctttgggctaagccggacatcccgcccaatacgttttcagtttcttctattccatgggtgcgcttttcaaacttcaatttaaaccttgataacagcgaacacttgctgccgattattacaaacgggaaatacttttcagaaggcagggaaacatttttgcccgtttccttgcaagttcaccatgcagtgtgtgacggctatcatgccggcgcttttataaacgagttggaacggcttgccgccgattgtgaggagtggcttgtgtgacagaggaaaggccgatatgattcggccttttttatatgtacttcttagcgggtctcttaacccccctcgaggtcgctgataaacagctgacatcaatatcctattttttcaaaaaatattttaaaaagttgttgacttaaaagaagctaaatgttatagtaataaaacagaatagtcttttaagtaagtctactctgaatttttttaaaaggagagggtaaagatgaaacaacaaaaacggctttacgcccgattgctgacgctgttatttgcgctcatcttcttgctgcctcattctgcagctagcgcagccgcaccgtttaacggtaccatgatgcagtattttgaatggtacttgccggatgatggcacgttatggaccaaagtggccaatgaagccaacaacttatccagccttggcatcaccgctctttggctgccgcccgcttacaaaggaacaagccgcagcgacgtagggtacggagtatacgacttgtatgacctcggcgaattcaatcaaaaagggaccgtccgcacaaaatatggaacaaaagctcaatatcttcaagccattcaagccgcccacgccgctggaatgcaagtgtacgccgatgtcgtgttcgaccataaaggcggcgctgacggcacggaatgggtggacgccgtcgaagtcaatccgtccgaccgcaaccaagaaatctcgggcacctatcaaatccaagcatggacgaaatttgattttcccgggcggggcaacacctactccagctttaagtggcgctggtaccattttgacggcgttgattgggacgaaagccgaaaattaagccgcatttacaaattcaggggcatcggcaaagcgtgggattggccggtagacacagaaaacggaaactatgactacttaatgtatgccgaccttgatatggatcatcccgaagtcgtgaccgagctgaaaaactgggggaaatggtatgtcaacacaacgaacattgatgggttccggcttgatgccgtcaagcatattaagttcagtttttttcctgattggttgtcgtatgtgcgttctcagactggcaagccgctatttaccgtcggggaatattggagctatgacatcaacaagttgcacaattacattacgaaaacaaacggaacgatgtctttgtttgatgccccgttacacaacaaattttataccgcttccaaatcagggggcgcatttgatatgcgcacgttaatgaccaatactctcatgaaagatcaaccgacattggccgtcaccttcgttgataatcatgacaccgaacccggccaagcgcttcagtcatgggtcgacccatggttcaaaccgttggcttacgcctttattctaactcggcaggaaggatacccgtgcgtcttttatggtgactattatggcattccacaatataacattccttcgctgaaaagcaaaatcgatccgctcctcatcgcgcgcagggattatgcttacggaacgcaacatgattatcttgatcactccgacatcatcgggtggacaagggaaggggtcactgaaaaaccaggatccgggctggccgcactgatcaccgatgggccgggaggaagcaaatggatgtacgttggcaaacaacacgctggaaaagtgttctatgaccttaccggcaaccggagtgacaccgtcaccatcaacagtgatggatggggggaattcaaagtcaatggcggttcggtttcggtttgggttcctagaaaaacgacctaaaagcttctcgaggttaacagaggacggatttcctgaaggaaatccgtttttttatttttaacatctctcactgctgtgtgattttactcacggcatttggaacgccggctctcaacaaactttctgtagtgaaaatcatgaaccaaacggatcgtcggcctgattaacagctgaaagctgccgatcacaaacatccatagtcccgccggcttcagttcctcggagaaaaagcagaagctcccgacaaggaataaaaggccgatgagaaaatcgtttaatgtatgtagaactttgtatctttttttgaaaaagagttcatatcgattgttattgttttgcggcattgcttgatcactccaatccttttatttaccctgccggaagccggagtgaaacgccggtatacataggatttatgaattaggaaaacatatggggaaataaaccatccaggagtgaaaaatatgcggttattcatatgtgcatcgtgcctgttcggcttgattgttccgtcatttgaaacgaaagcgctgacgtttgaagaattgccggttaaacaagcttcaaaacaatgggaagttcaaatcggtaaagccgaagccggaaacggaatggcgaaaccggaaaaaggagcgtttcatacttatgctgtcgaaatcaaaaacattggacacgatgtggcttcggcggaaatttttgtctatcggaacgagcctaattcttcaacgaaattttcgctttggaacattcctcacgaaaatccggtttctttagccaaaagcttaaatcacggaagctctgtcaagcaccgcaatctgcttatggcagagaatgcgaccgaattggaagtggacatgatttggacggaaaaaggaagcgaaggcagacttttaaaggaaacgttcattttcaagggagatgaatcatgaagaaaaaatggccgttcatcgtcaacggtctttttttaatgacttaggcagccgatcgttcggccatacgatatcgaagcgacctcgaaccagcagagctcgtcacaaaacatttgcatttaaagaaaaatacaggatgttttcaccaatatttttctcaatgatgatacactattgacaagctgctactttgggagggtgtttccatagatgccgatgaagcaaaaacaccaaatgtgtcatgagagctctctctaatcgatataaaagtagggtgaaccggggttgtcaatctgtaaaagatctttttttatcccgtgatacgcttttggaattctgaatcttcaagaaagtccccagccttttgctgatcaatcgagaacaaaggatgatacatatgaaaagaatagataaaatctaccatcagctgctggataattttcgcgaaaagaatatcaatcagcttttaaagatacaagggaattcggctaaagaaatcgccgggcagctgcaaatggagcgttccaatgtcagctttgaattaaacaatctggttcgggccaaaaaggtgatcaagattaaaacgttccccgtccgctacatcccggtggaaattgttgaaaacgtcttgaacatcaaatggaattcagagttgatggaggttgaagaactgaggcggctggctgacggccaaaaaaagccggcgcgcaatatatccgccgatcccctcgagctcatgatcggggctaaagggagcttgaaaaaggcaatttctcaggcgaaagcggcagtcttttatcctccgcacggcttgcatatgctgctgctcgggccgacgggttcggggaaatcgctgtttgcgaatcggatctaccagttcgccgtttattctgacatattgaagcccgattccccgttcatcacattcaactgtgcag

SEQ ID NO: 66 - DNA, 1703 bp, Bacillus licheniformis
ggctatgacgaaacgattgcagcctatgaggcgagtctcgaaaagctcggacttgactaccttgatttatacctgatccactggcctgttgaaggacgctacaaagcggcgtggaaagcgcttgaaacactttatgaacaaggacgcgtaaaagcaatcggagtgagcaattttcagattcaccatctggaagacttgctgaaagatgccgccgtcaaaccggcgatcaaccaggttgagtatcatccgcggctgacgcagaaagagctgcaagcgttttgccgtgcgcacggcatccagctgcaagcatggtcgccgctgatgcaaggccaattgctcagccatccactgctgaaagatatcgcggacaagtacggcaagacaccggcccaagtcattttgcgctgggatttgcaaaacggggtcgttacgattccgaagtcgactaaagcggagcggattgcccaaaacgcggacatatttgattttgaactgaccaccgaggaaatgaagcaaattgacgcgctgaatgaaaacacccgtgtcggccctgatcccgataactttgacttttaacaaaacggccccgttcgacattcgaacggggctttaattgaattgtgcggttacaccgccggactccatcatcatcagttcttttttcatatccaatccgccccggtatcccgtgagctgcccgcttttaccgataacccgatggcaaggcaccaccattaacagcggatttgcgccgatcgccgcgcctactgcccgcacagcggcctgcttttcaatatgctcggcgatatcggaataggagcaagtgctgccgtaagggatttcggagagcgccttccacactgccagctgaaaaggcgtgccggcaaggtcgacaggaaagctgaaatgagttcgcttgccgttcaaatacgcctgcagctgctcggcgtattctgccaatcctttgtcatcccgaatgaaaactggctgtgtaaatcttttttcagcccaagcggccaaatcctcgaagccttgattccatccccctgtaaaacagagcccgcgggcagtcgccccaatgtgaatctgccaacctcggcaaataagcgtacgccagtatacgatttgatcgtccatatgtttacctccgtttcatttgccggtacgacgtcggcgattgcccagtcttctttttaaacaaagaggcaaaatattccgcattcgcaatgcctaccattgaagcgatttctgcgatcgatcgttctgaatgagcaagcaaatcgaccgctttctcaatccttttctgcaggatgtattctgccggcgagacgcctttgattcgtttaaatgtccgctgcaggtgaaaagggctgatatggcacctgtcagccaaagcttgcagagacagcggatcgcgataagattcctcgatgatttccaccacacgctgtgccagctcttcatccggcagcagcgccccggccggattgcagcgtttgcaggggcggtacccttctgataaagcatcttttgcattgaaaaagatctgcacattgtcgatttgcggaactctcgatttgcaggaagggcggcaaaatatgccggtcgttttgaccgcgtaataaaaaactccgtcataggcggaatcgttttccgtaatcgcccgccacatttcaggcgtcaatcgtgatttgctgttcata

SEQ ID NO: 67 - DNA, 937 bp, Bacillus licheniformis
atcttcaccccgatctatgtcagtataacctatatgacagccggaggtggagaggcggagaacggcacagcaagaagacaaagaagaagagagactgttgcctggacctccgaaacgcgctacaattcatttacaacacaggatggggtgagaatattgccggaatcagtgaagcaggcctcctaaaataaaaatctatattttaggaggtaaaacatgaattttcaaacaatcgagcttgacacatggtatagaaaatcttattttgaccattacatgaaggaagcgaaatgttctttcagcatcacggcaaacgtcaatgtgacaaatttgctcgccgtgctcaagaaaaagaagctcaagctgtatccggcttttatttatatcgtatcaagggtcattcattcgcgccctgagtttagaacaacgtttgatgacaaaggacagctgggttattgggaacaaatgcatccgtgctatgcgatttttcatcaggacgaccaaacgttttccgccctctggacggaatactcagacgatttttcgcagttttatcatcaatatcttctggacgccgagcgctttggagacaaaaggggcctttgggctaagccggacatcccgcccaatacgttttcagtttcttctattccatgggtgcgcttttcaaacttcaatttaaaccttgataacagcgaacacttgctgccgattattacaaacgggaaatacttttcagaaggcagggaaacatttttgcccgtttccttgcaagttcaccatgcagtgtgtgacggctatcatgccggcgcttttataaacgagttggaacggcttgccgccgattgtgaggagtggcttgtgtgacagaggaaaggccgatatgattcggccttttttatatgtacttcttagcgggtctcttaacccccctcga

SEQ ID NO: 68 - DNA, 95 bp, Artificial Sequence
  spoVGrrnIp hybrid promoter
gtcgctgataaacagctgacatcaatatcctattttttcaaaaaatattttaaaaagttgttgacttaaaagaagctaaatgttatagtaataaa

SEQ ID NO: 69 - DNA, 87 bp, Bacillus licheniformis
atgaaacaacaaaaacggctttacgcccgattgctgacgctgttatttgcgctcatcttcttgctgcctcattctgcagctagcgca

SEQ ID NO: 70 - DNA, 1461 bp, G. stearothermophilus
gccgcaccgtttaacggtaccatgatgcagtattttgaatggtacttgccggatgatggcacgttatggaccaaagtggccaatgaagccaacaacttatccagccttggcatcaccgctctttggctgccgcccgcttacaaaggaacaagccgcagcgacgtagggtacggagtatacgacttgtatgacctcggcgaattcaatcaaaaagggaccgtccgcacaaaatatggaacaaaagctcaatatcttcaagccattcaagccgcccacgccgctggaatgcaagtgtacgccgatgtcgtgttcgaccataaaggcggcgctgacggcacggaatgggtggacgccgtcgaagtcaatccgtccgaccgcaaccaagaaatctcgggcacctatcaaatccaagcatggacgaaatttgattttcccgggcggggcaacacctactccagctttaagtggcgctggtaccattttgacggcgttgattgggacgaaagccgaaaattaagccgcatttacaaattcaggggcatcggcaaagcgtgggattggccggtagacacagaaaacggaaactatgactacttaatgtatgccgaccttgatatggatcatcccgaagtcgtgaccgagctgaaaaactgggggaaatggtatgtcaacacaacgaacattgatgggttccggcttgatgccgtcaagcatattaagttcagtttttttcctgattggttgtcgtatgtgcgttctcagactggcaagccgctatttaccgtcggggaatattggagctatgacatcaacaagttgcacaattacattacgaaaacaaacggaacgatgtctttgtttgatgccccgttacacaacaaattttataccgcttccaaatcagggggcgcatttgatatgcgcacgttaatgaccaatactctcatgaaagatcaaccgacattggccgtcaccttcgttgataatcatgacaccgaacccggccaagcgcttcagtcatgggtcgacccatggttcaaaccgttggcttacgcctttattctaactcggcaggaaggatacccgtgcgtcttttatggtgactattatggcattccacaatataacattccttcgctgaaaagcaaaatcgatccgctcctcatcgcgcgcagggattatgcttacggaacgcaacatgattatcttgatcactccgacatcatcgggtggacaagggaaggggtcactgaaaaaccaggatccgggctggccgcactgatcaccgatgggccgggaggaagcaaatggatgtacgttggcaaacaacacgctggaaaagtgttctatgaccttaccggcaaccggagtgacaccgtcaccatcaacagtgatggatggggggaattcaaagtcaatggcggttcggtttcggtttgggttcctagaaaaacgacctaa

SEQ ID NO: 71 - DNA, 34 bp, Bacillus licheniformis
cggatttcctgaaggaaatccgtttttttatttt

SEQ ID NO: 72 - DNA, 1809 bp, Bacillus licheniformis
taacatctctcactgctgtgtgattttactcacggcatttggaacgccggctctcaacaaactttctgtagtgaaaatcatgaaccaaacggatcgtcggcctgattaacagctgaaagctgccgatcacaaacatccatagtcccgccggcttcagttcctcggagaaaaagcagaagctcccgacaaggaataaaaggccgatgagaaaatcgtttaatgtatgtagaactttgtatctttttttgaaaaagagttcatatcgattgttattgttttgcggcattgcttgatcactccaatccttttatttaccctgccggaagccggagtgaaacgccggtatacataggatttatgaattaggaaaacatatggggaaataaaccatccaggagtgaaaaatatgcggttattcatatgtgcatcgtgcctgttcggcttgattgttccgtcatttgaaacgaaagcgctgacgtttgaagaattgccggttaaacaagcttcaaaacaatgggaagttcaaatcggtaaagccgaagccggaaacggaatggcgaaaccggaaaaaggagcgtttcatacttatgctgtcgaaatcaaaaacattggacacgatgtggcttcggcggaaatttttgtctatcggaacgagcctaattcttcaacgaaattttcgctttggaacattcctcacgaaaatccggtttctttagccaaaagcttaaatcacggaagctctgtcaagcaccgcaatctgcttatggcagagaatgcgaccgaattggaagtggacatgatttggacggaaaaaggaagcgaaggcagacttttaaaggaaacgttcattttcaagggagatgaatcatgaagaaaaaatggccgttcatcgtcaacggtctttttttaatgacttaggcagccgatcgttcggccatacgatatcgaagcgacctcgaaccagcagagctcgtcacaaaacatttgcatttaaagaaaaatacaggatgttttcaccaatatttttctcaatgatgatacactattgacaagctgctactttgggagggtgtttccatagatgccgatgaagcaaaaacaccaaatgtgtcatgagagctctctctaatcgatataaaagtagggtgaaccggggttgtcaatctgtaaaagatctttttttatcccgtgatacgcttttggaattctgaatcttcaagaaagtccccagccttttgctgatcaatcgagaacaaaggatgatacatatgaaaagaatagataaaatctaccatcagctgctggataattttcgcgaaaagaatatcaatcagcttttaaagatacaagggaattcggctaaagaaatcgccgggcagctgcaaatggagcgttccaatgtcagctttgaattaaacaatctggttcgggccaaaaaggtgatcaagattaaaacgttccccgtccgctacatcccggtggaaattgttgaaaacgtcttgaacatcaaatggaattcagagttgatggaggttgaagaactgaggcggctggctgacggccaaaaaaagccggcgcgcaatatatccgccgatcccctcgagctcatgatcggggctaaagggagcttgaaaaaggcaatttctcaggcgaaagcggcagtcttttatcctccgcacggcttgcatatgctgctgctcgggccgacgggttcggggaaatcgctgtttgcgaatcggatctaccagttcgccgtttattctgacatattgaagcccgattccccgttcatcacattcaactgtgcag

SEQ ID NO: 73 - protein, 486 aa, G. stearothermophilus
AAPFNGTMMQYFEWYLPDDGTLWTKVANEANNLSSLGITALWLPPAYKGTSRSDVGYGVYDLYDLGEFNQKGTVRTKYGTKAQYLQAIQAAHAAGMQVYADVVFDHKGGADGTEWVDAVEVNPSDRNQEISGTYQIQAWTKFDFPGRGNTYSSFKWRWYHFDGVDWDESRKLSRIYKFRGIGKAWDWPVDTENGNYDYLMYADLDMDHPEVVTELKNWGKWYVNTTNIDGFRLDAVKHIKFSFFPDWLSYVRSQTGKPLFTVGEYWSYDINKLHNYITKTNGTMSLFDAPLHNKFYTASKSGGAFDMRTLMTNTLMKDQPTLAVTFVDNHDTEPGQALQSWVDPWFKPLAYAFILTRQEGYPCVFYGDYYGIPQYNIPSLKSKIDPLLIARRDYAYGTQHDYLDHSDIIGWTREGVTEKPGSGLAALITDGPGGSKWMYVGKQHAGKVFYDLTGNRSDTVTINSDGWGEFKVNGGSVSVWVPRKTT

SEQ ID NO: 74 - DNA, 1967 bp, Artificial Sequence
  catH locus WT construct
tgtgtgacggctatcatgccggcgcttttataaacgagttggaacggcttgccgccgattgtgaggagtggcttgtgtgacagaggaaaggccgatatgattcggccttttttatatgtacttcttagcgggtctcttaacccccctcgaggtcgctgataaacagctgacatcaatatcctattttttcaaaaaatattttaaaaagttgttgacttaaaagaagctaaatgttatagtaataaaacagaatagtcttttaagtaagtctactctgaatttttttaaaaggagagggtaaagaatgaaacaacaaaaacggctttacgcccgattgctgacgctgttatttgcgctcatcttcttgctgcctcattctgcagctagcgcagccgcaccgtttaacggtaccatgatgcagtattttgaatggtacttgccggatgatggcacgttatggaccaaagtggccaatgaagccaacaacttatccagccttggcatcaccgctctttggctgccgcccgcttacaaaggaacaagccgcagcgacgtagggtacggagtatacgacttgtatgacctcggcgaattcaatcaaaaagggaccgtccgcacaaaatatggaacaaaagctcaatatcttcaagccattcaagccgcccacgccgctggaatgcaagtgtacgccgatgtcgtgttcgaccataaaggcggcgctgacggcacggaatgggtggacgccgtcgaagtcaatccgtccgaccgcaaccaagaaatctcgggcacctatcaaatccaagcatggacgaaatttgattttcccgggcggggcaacacctactccagctttaagtggcgctggtaccattttgacggcgttgattgggacgaaagccgaaaattaagccgcatttacaaattcaggggcatcggcaaagcgtgggattggccggtagacacagaaaacggaaactatgactacttaatgtatgccgaccttgatatggatcatcccgaagtcgtgaccgagctgaaaaactgggggaaatggtatgtcaacacaacgaacattgatgggttccggcttgatgccgtcaagcatattaagttcagtttttttcctgattggttgtcgtatgtgcgttctcagactggcaagccgctatttaccgtcggggaatattggagctatgacatcaacaagttgcacaattacattacgaaaacaaacggaacgatgtctttgtttgatgccccgttacacaacaaattttataccgcttccaaatcagggggcgcatttgatatgcgcacgttaatgaccaatactctcatgaaagatcaaccgacattggccgtcaccttcgttgataatcatgacaccgaacccggccaagcgcttcagtcatgggtcgacccatggttcaaaccgttggcttacgcctttattctaactcggcaggaaggatacccgtgcgtcttttatggtgactattatggcattccacaatataacattccttcgctgaaaagcaaaatcgatccgctcctcatcgcgcgcagggattatgcttacggaacgcaacatgattatcttgatcactccgacatcatcgggtggacaagggaaggggtcactgaaaaaccaggatccgggctggccgcactgatcaccgatgggccgggaggaagcaaatggatgtacgttggcaaacaacacgctggaaaagtgttctatgaccttaccggcaaccggagtgacaccgtcaccatcaacagtgatggatggggggaattcaaagtcaatggcggttcggtttcggtttgggttcctagaaaaacgacctaaaagcttctcgaggttaacagaggacggatttcctgaaggaaatccgtttttttatttttaacatctctcactgctgtgtgattttactcacggcatttggaacgccggctctcaa

SEQ ID NO: 75 - DNA, 1966 bp, Artificial Sequence
  catH locus mod 5'-UTR construct
tgtgtgacggctatcatgccggcgcttttataaacgagttggaacggcttgccgccgattgtgaggagtggcttgtgtgacagaggaaaggccgatatgattcggccttttttatatgtacttcttagcgggtctcttaacccccctcgaggtcgctgataaacagctgacatcaatatcctattttttcaaaaaatattttaaaaagttgttgacttaaaagaagctaaatgttatagtaataaaacagaatagtcttttaagtaagtctactctgaatttttttaaaaggagagggtaaagatgaaacaacaaaaacggctttacgcccgattgctgacgctgttatttgcgctcatcttcttgctgcctcattctgcagctagcgcagccgcaccgtttaacggtaccatgatgcagtattttgaatggtacttgccggatgatggcacgttatggaccaaagtggccaatgaagccaacaacttatccagccttggcatcaccgctctttggctgccgcccgcttacaaaggaacaagccgcagcgacgtagggtacggagtatacgacttgtatgacctcggcgaattcaatcaaaaagggaccgtccgcacaaaatatggaacaaaagctcaatatcttcaagccattcaagccgcccacgccgctggaatgcaagtgtacgccgatgtcgtgttcgaccataaaggcggcgctgacggcacggaatgggtggacgccgtcgaagtcaatccgtccgaccgcaaccaagaaatctcgggcacctatcaaatccaagcatggacgaaatttgattttcccgggcggggcaacacctactccagctttaagtggcgctggtaccattttgacggcgttgattgggacgaaagccgaaaattaagccgcatttacaaattcaggggcatcggcaaagcgtgggattggccggtagacacagaaaacggaaactatgactacttaatgtatgccgaccttgatatggatcatcccgaagtcgtgaccgagctgaaaaactgggggaaatggtatgtcaacacaacgaacattgatgggttccggcttgatgccgtcaagcatattaagttcagtttttttcctgattggttgtcgtatgtgcgttctcagactggcaagccgctatttaccgtcggggaatattggagctatgacatcaacaagttgcacaattacattacgaaaacaaacggaacgatgtctttgtttgatgccccgttacacaacaaattttataccgcttccaaatcagggggcgcatttgatatgcgcacgttaatgaccaatactctcatgaaagatcaaccgacattggccgtcaccttcgttgataatcatgacaccgaacccggccaagcgcttcagtcatgggtcgacccatggttcaaaccgttggcttacgcctttattctaactcggcaggaaggatacccgtgcgtcttttatggtgactattatggcattccacaatataacattccttcgctgaaaagcaaaatcgatccgctcctcatcgcgcgcagggattatgcttacggaacgcaacatgattatcttgatcactccgacatcatcgggtggacaagggaaggggtcactgaaaaaccaggatccgggctggccgcactgatcaccgatgggccgggaggaagcaaatggatgtacgttggcaaacaacacgctggaaaagtgttctatgaccttaccggcaaccggagtgacaccgtcaccatcaacagtgatggatggggggaattcaaagtcaatggcggttcggtttcggtttgggttcctagaaaaacgacctaaaagcttctcgaggttaacagaggacggatttcctgaaggaaatccgtttttttatttttaacatctctcactgctgtgtgattttactcacggcatttggaacgccggctctcaa

SEQ ID NO: 76 - DNA, 20 bp, Artificial Sequence
  catH locus forward primer
tgtgtgacggctatcatgcc

SEQ ID NO: 77 - DNA, 17 bp, Artificial Sequence
  catH locus reverse primer
ttgagagccggcgttcc

SEQ ID NO: 78 - DNA, 20 bp, Artificial Sequence
  catH forward sequencing primer 1
aacgagttggaacggcttgc

SEQ ID NO: 79 - DNA, 20 bp, Artificial Sequence
  catH forward sequencing primer 2
ggcaacacctactccagctt

SEQ ID NO: 80 - DNA, 20 bp, Artificial Sequence
  catH forward sequencing primer 3
gatcactccgacatcatcgg

SEQ ID NO: 81 - DNA, 1205 bp, Bacillus licheniformis
catcaatctttttccagacagtgatcaaaattcgacatttttcatcaaaaacgtcaaaataaattgacgcgctttcatgagttttgtacgatatgagagattgatgacaaaaaggagctgaggatcgtgaacagatcctttaccgttgaaaaggtactcaacaacaacgttttaatcgctctccatgatgattacagagaagttgtcttgattggcaaaggaatcggttttggtaaaaagcgcggagatcttatcgaacatgagaactacgaaaaaatgtttatcctggaaaatgataaggaacaatcgcagtataagaagctcctcacttatgtcgatgaaaaaatggttgatatcgccaatgatgtcatctaccatatcgcgcaaaaaatcggccagccgctgaacgaacacattcatgtcgccctgacggaccatatcgcatttgcagttaagcgtctagaaaagggatttgatatgaaaaatccgtttttgcttgagacggaatcgctttatccgaaggaatacgaagtcgccaaggaagccgtcgatatgattaatgaaaaatccgacattcagctgcctgaaggtgaaatcgggttcatcgcgcttcatatccacagtgcgatgacaaaccgcccgctttctgaagtcaatcagcattcacaactgatctccaggcttgtccaggtcatcgaagattcattccagatgcaagtcaacagggaaagcgtgaactatttgcggctgatcaggcacttgcgctttacgattgacaggataaaacgggacgagccgattcaggaaccggaaaaattaatgttgttgttgaaaacggaatatccgctgtgttacaatactgcttggaagatgatcaagatcttgcagcaagcgctcaagaaaccggttcatgaggcagaagccgtttatttgacattgcatttgtaccgtttgactaataaaatttcataacgcctttataacgtgttactgattcgatcaggcatgagtgaaaaaaggggagaaatgaagacgctgtcttttgtttcttagtgtacccgctttcaccatgccttttttgtcgttctaaaggcgaaatgtaaacggtttatttagatgaaaaagcagtcttttgaacgaagttgtcatgaatttttgctgtaaggtcaaactattcttagagggggttaaaaaatgtttaaatc

SEQ ID NO: 82 - protein, 281 aa, Bacillus licheniformis
VNRSFTVEKVLNNNVLIALHDDYREVVLIGKGIGFGKKRGDLIEHENYEKMFILENDKEQSQYKKLLTYVDEKMVDIANDVIYHIAQKIGQPLNEHIHVALTDHIAFAVKRLEKGFDMKNPFLLETESLYPKEYEVAKEAVDMINEKSDIQLPEGEIGFIALHIHSAMTNRPLSEVNQHSQLISRLVQVIEDSFQMQVNRESVNYLRLIRHLRFTIDRIKRDEPIQEPEKLMLLLKTEYPLCYNTAWKMIKILQQALKKPVHEAEAVYLTLHLYRLTNKIS

SEQ ID NO: 83 - protein, 140 aa, Bacillus licheniformis
MAMTRFGERLKELREQRSLSVNQLAMYAGVSAAAISRAAAISRIENGHRGVPKPATIRKLAEALKMPYEQLMDIAGYMRADEIREQPRGYVTMQEIAAKHGVEDLWLFKPEKWDCLSREDLLNLEQYFHFLVNEAKKRQS

SEQ ID NO: 84 - protein, 134 aa, Bacillus licheniformis
MAMTRFGERLKELREQRSLSVNQLAMYAGVSAAAISRIENGHRGVPKPATIRKLAEALKMPYEQLMDIAGYMRADEIREQPRGYVTMQEIAAKHGVEDLWLFKPEKWDCLSREDLLNLEQYFHFLVNEAKKRQS